European Patent Specification EP 3 583 126 B1, published August 27, 2025. Title: MULTISPECIFIC BINDING MOLECULES HAVING SPECIFICITY TO DYSTROGLYCAN AND LAMININ-2. Applicant: Sanofi BEIL, Christian BRONDYK, William CHEN, Yangde CHEN, Seng H. CONNORS, Timothy D. DEVAUD, Catherine HOFFMANN, Dietmar LANGE, Christian MAGNAY, Maureen MAGNAY, Tristan PRADES, Catherine RAO, Ercole SEVIGNY, Leila ZHU, Yunxiang WEI, Ronnie ZHAO, Hongmei ZHU, Yunxiang. Application Not Yet Assigned. The sequence listing filed with the application follows.

SEQUENCE LISTING (534 sequences)

SEQ ID NO: 1 - protein, 8 aa, Artificial Sequence
  Synthetic Construct
GFTFTDSV

SEQ ID NO: 2 - protein, 8 aa, Artificial Sequence
  Synthetic Construct
GFTFSSYA

SEQ ID NO: 3 - protein, 8 aa, Artificial Sequence
  Synthetic Construct
GYSFSNYW

SEQ ID NO: 4 - protein, 8 aa, Artificial Sequence
  Synthetic Construct
GFNIKDTY

SEQ ID NO: 5 - protein, 8 aa, Artificial Sequence
  Synthetic Construct
GYTFTTYY

SEQ ID NO: 6 - protein, 8 aa, Artificial Sequence
  Synthetic Construct
GFTFSSYG

SEQ ID NO: 7 - protein, 8 aa, Artificial Sequence
  Synthetic Construct
GYSFTSYW

SEQ ID NO: 8 - protein, 8 aa, Artificial Sequence
  Synthetic Construct
GYSFTSYW

SEQ ID NO: 9 - protein, 8 aa, Artificial Sequence
  Synthetic Construct
IYPGSGSI

SEQ ID NO: 10 - protein, 8 aa, Artificial Sequence
  Synthetic Construct
IYPGSGNF

SEQ ID NO: 11 - protein, 8 aa, Artificial Sequence
  Synthetic Construct
ISGSGGST

SEQ ID NO: 12 - protein, 8 aa, Artificial Sequence
  Synthetic Construct
IYPGDSDT

SEQ ID NO: 13 - protein, 8 aa, Artificial Sequence
  Synthetic Construct
IDPANGNT

SEQ ID NO: 14 - protein, 8 aa, Artificial Sequence
  Synthetic Construct
INPSAGNT

SEQ ID NO: 15 - protein, 8 aa, Artificial Sequence
  Synthetic Construct
IWYDGSNK

SEQ ID NO: 16 - protein, 8 aa, Artificial Sequence
  Synthetic Construct
IYPGDSDT

SEQ ID NO: 17 - protein, 8 aa, Artificial Sequence
  Synthetic Construct
IYPGDSDT

SEQ ID NO: 18 - protein, 6 aa, Artificial Sequence
  Synthetic Construct
AMRRSY

SEQ ID NO: 19 - protein, 6 aa, Artificial Sequence
  Synthetic Construct
AMRRSS

SEQ ID NO: 20 - protein, 18 aa, Artificial Sequence
  Synthetic Construct
ARLGYCSSTSCYLSAFDI

SEQ ID NO: 21 - protein, 13 aa, Artificial Sequence
  Synthetic Construct
RVIINGTTSGFDY

SEQ ID NO: 22 - protein, 10 aa, Artificial Sequence
  Synthetic Construct
GRSGGNYVGY

SEQ ID NO: 23 - protein, 10 aa, Artificial Sequence
  Synthetic Construct
GRSRGNYFDY

SEQ ID NO: 24 - protein, 6 aa, Artificial Sequence
  Synthetic Construct
ARELDI

SEQ ID NO: 25 - protein, 13 aa, Artificial Sequence
  Synthetic Construct
AREGMVRGALFDY

SEQ ID NO: 26 - protein, 12 aa, Artificial Sequence
  Synthetic Construct
ARQLRDYYGMDV

SEQ ID NO: 27 - protein, 12 aa, Artificial Sequence
  Synthetic Construct
ARQLRDYYSMDV

SEQ ID NO: 28 - protein, 11 aa, Artificial Sequence
  Synthetic Construct
QSIVHSNGNTY

SEQ ID NO: 29 - protein, 11 aa, Artificial Sequence
  Synthetic Construct
QTIVHSNSKTY

SEQ ID NO: 30 - protein, 6 aa, Artificial Sequence
  Synthetic Construct
QSISSW

SEQ ID NO: 31 - protein, 6 aa, Artificial Sequence
  Synthetic Construct
QSVSSN

SEQ ID NO: 32 - protein, 12 aa, Artificial Sequence
  Synthetic Construct
QSLLDSGNQKNY

SEQ ID NO: 33 - protein, 10 aa, Artificial Sequence
  Synthetic Construct
QSLKSNQKNY

SEQ ID NO: 34 - protein, 6 aa, Artificial Sequence
  Synthetic Construct
QDIRND

SEQ ID NO: 35 - protein, 7 aa, Artificial Sequence
  Synthetic Construct
QSVSSSY

SEQ ID NO: 36 - protein, 7 aa, Artificial Sequence
  Synthetic Construct
QTISSNY

SEQ ID NO: 37 - protein, 7 aa, Artificial Sequence
  Synthetic Construct
QSVSSSY

SEQ ID NO: 38 - protein, 3 aa, Artificial Sequence
  Synthetic Construct
KVS

SEQ ID NO: 39 - protein, 3 aa, Artificial Sequence
  Synthetic Construct
DAS

SEQ ID NO: 40 - protein, 3 aa, Artificial Sequence
  Synthetic Construct
GAS

SEQ ID NO: 41 - protein, 3 aa, Artificial Sequence
  Synthetic Construct
WAS

SEQ ID NO: 42 - protein, 3 aa, Artificial Sequence
  Synthetic Construct
AAS

SEQ ID NO: 43 - protein, 9 aa, Artificial Sequence
  Synthetic Construct
FQGSHVPLT

SEQ ID NO: 44 - protein, 9 aa, Artificial Sequence
  Synthetic Construct
QQYNSYPLT

SEQ ID NO: 45 - protein, 9 aa, Artificial Sequence
  Synthetic Construct
QHYNNLPLT

SEQ ID NO: 46 - protein, 9 aa, Artificial Sequence
  Synthetic Construct
QQYYTYPWT

SEQ ID NO: 47 - protein, 9 aa, Artificial Sequence
  Synthetic Construct
LQDFNFPFT

SEQ ID NO: 48 - protein, 9 aa, Artificial Sequence
  Synthetic Construct
QQDYNLPYT

SEQ ID NO: 49 - protein, 9 aa, Artificial Sequence
  Synthetic Construct
QQDYNLPRT

SEQ ID NO: 50 - protein, 9 aa, Artificial Sequence
  Synthetic Construct
QQDYNLPRT

SEQ ID NO: 51 - protein, 8 aa, Artificial Sequence
  Synthetic Construct
GYTFTSYN

SEQ ID NO: 52 - protein, 8 aa, Artificial Sequence
  Synthetic Construct
GFTFSSYT

SEQ ID NO: 53 - protein, 8 aa, Artificial Sequence
  Synthetic Construct
GFTFSSYT

SEQ ID NO: 54 - protein, 8 aa, Artificial Sequence
  Synthetic Construct
GYSFTSYW

SEQ ID NO: 55 - protein, 8 aa, Artificial Sequence
  Synthetic Construct
GFTFDDYG

SEQ ID NO: 56 - protein, 8 aa, Artificial Sequence
  Synthetic Construct
INPYNDGT

SEQ ID NO: 57 - protein, 8 aa, Artificial Sequence
  Synthetic Construct
ISSGGGNT

SEQ ID NO: 58 - protein, 8 aa, Artificial Sequence
  Synthetic Construct
ISSGGDNT

SEQ ID NO: 59 - protein, 8 aa, Artificial Sequence
  Synthetic Construct
IYPGDSDT

SEQ ID NO: 60 - protein, 8 aa, Artificial Sequence
  Synthetic Construct
INWNGGST

SEQ ID NO: 61 - protein, 7 aa, Artificial Sequence
  Synthetic Construct
AIYGNSY

SEQ ID NO: 62 - protein, 11 aa, Artificial Sequence
  Synthetic Construct
ARFDYGSSLDS

SEQ ID NO: 63 - protein, 11 aa, Artificial Sequence
  Synthetic Construct
ARFDYGSSLDC

SEQ ID NO: 64 - protein, 13 aa, Artificial Sequence
  Synthetic Construct
ARRGYRSSWYFDY

SEQ ID NO: 65 - protein, 11 aa, Artificial Sequence
  Synthetic Construct
AREGGELLMDY

SEQ ID NO: 66 - protein, 11 aa, Artificial Sequence
  Synthetic Construct
KSLLHSNGNTY

SEQ ID NO: 67 - protein, 6 aa, Artificial Sequence
  Synthetic Construct
QSISNN

SEQ ID NO: 68 - protein, 6 aa, Artificial Sequence
  Synthetic Construct
QSISNY

SEQ ID NO: 69 - protein, 6 aa, Artificial Sequence
  Synthetic Construct
QGIRND

SEQ ID NO: 70 - protein, 6 aa, Artificial Sequence
  Synthetic Construct
QSVSTY

SEQ ID NO: 71 - protein, 3 aa, Artificial Sequence
  Synthetic Construct
YMS

SEQ ID NO: 72 - protein, 3 aa, Artificial Sequence
  Synthetic Construct
YAS

SEQ ID NO: 73 - protein, 3 aa, Artificial Sequence
  Synthetic Construct
YAS

SEQ ID NO: 74 - protein, 3 aa, Artificial Sequence
  Synthetic Construct
AAS

SEQ ID NO: 75 - protein, 3 aa, Artificial Sequence
  Synthetic Construct
DAS

SEQ ID NO: 76 - protein, 9 aa, Artificial Sequence
  Synthetic Construct
MQGLEYPYT

SEQ ID NO: 77 - protein, 9 aa, Artificial Sequence
  Synthetic Construct
QQSKNWPRT

SEQ ID NO: 78 - protein, 9 aa, Artificial Sequence
  Synthetic Construct
QQSKSWPRT

SEQ ID NO: 79 - protein, 9 aa, Artificial Sequence
  Synthetic Construct
LQDYNYPLT

SEQ ID NO: 80 - protein, 9 aa, Artificial Sequence
  Synthetic Construct
QQRSNWPPT

SEQ ID NO: 81 - protein, 8 aa, Artificial Sequence
  Synthetic Construct
GFTFSHYS

SEQ ID NO: 82 - protein, 8 aa, Artificial Sequence
  Synthetic Construct
GFTFSWYP

SEQ ID NO: 83 - protein, 8 aa, Artificial Sequence
  Synthetic Construct
GFTFSDYE

SEQ ID NO: 84 - protein, 8 aa, Artificial Sequence
  Synthetic Construct
GFTFSYYD

SEQ ID NO: 85 - protein, 8 aa, Artificial Sequence
  Synthetic Construct
GFTFSHYQ

SEQ ID NO: 86 - protein, 8 aa, Artificial Sequence
  Synthetic Construct
GYTFTGYY

SEQ ID NO: 87 - protein, 8 aa, Artificial Sequence
  Synthetic Construct
GNTFTGYY

SEQ ID NO: 88 - protein, 8 aa, Artificial Sequence
  Synthetic Construct
GFTFSSYG

SEQ ID NO: 89 - protein, 8 aa, Artificial Sequence
  Synthetic Construct
GFTFSSYA

SEQ ID NO: 90 - protein, 8 aa, Artificial Sequence
  Synthetic Construct
GFTFSGYG

SEQ ID NO: 91 - protein, 8 aa, Artificial Sequence
  Synthetic Construct
GFTFSSFG

SEQ ID NO: 92 - protein, 8 aa, Artificial Sequence
  Synthetic Construct
GFTFNRFV

SEQ ID NO: 93 - protein, 8 aa, Artificial Sequence
  Synthetic Construct
GGSFSGYY

SEQ ID NO: 94 - protein, 8 aa, Artificial Sequence
  Synthetic Construct
GYTFTSYE

SEQ ID NO: 95 - protein, 8 aa, Artificial Sequence
  Synthetic Construct
GFTFSRYA

SEQ ID NO: 96 - protein, 7 aa, Artificial Sequence
  Synthetic Construct
IYPSGGT

SEQ ID NO: 97 - protein, 8 aa, Artificial Sequence
  Synthetic Construct
IYPSGGTT

SEQ ID NO: 98 - protein, 8 aa, Artificial Sequence
  Synthetic Construct
IWPSGGLT

SEQ ID NO: 99 - protein, 8 aa, Artificial Sequence
  Synthetic Construct
IYSSGGHT

SEQ ID NO: 100 - protein, 8 aa, Artificial Sequence
  Synthetic Construct
ISPSGGFT

SEQ ID NO: 101 - protein, 8 aa, Artificial Sequence
  Synthetic Construct
INPNSGGT

SEQ ID NO: 102 - protein, 8 aa, Artificial Sequence
  Synthetic Construct
IKPSTGDT

SEQ ID NO: 103 - protein, 8 aa, Artificial Sequence
  Synthetic Construct
IWYDGSNK

SEQ ID NO: 104 - protein, 8 aa, Artificial Sequence
  Synthetic Construct
ISGRGGSP

SEQ ID NO: 105 - protein, 8 aa, Artificial Sequence
  Synthetic Construct
IWSDGSNR

SEQ ID NO: 106 - protein, 8 aa, Artificial Sequence
  Synthetic Construct
IYYDGSNK

SEQ ID NO: 107 - protein, 8 aa, Artificial Sequence
  Synthetic Construct
ISGSGGST

SEQ ID NO: 108 - protein, 7 aa, Artificial Sequence
  Synthetic Construct
INHSGGT

SEQ ID NO: 109 - protein, 8 aa, Artificial Sequence
  Synthetic Construct
IYPRDGDT

SEQ ID NO: 110 - protein, 8 aa, Artificial Sequence
  Synthetic Construct
ISSGGDYI

SEQ ID NO: 111 - protein, 19 aa, Artificial Sequence
  Synthetic Construct
ARHWRGYSSSWYHPAYFDY

SEQ ID NO: 112 - protein, 19 aa, Artificial Sequence
  Synthetic Construct
ARSYYYDSSGYYSHDAFDI

SEQ ID NO: 113 - protein, 15 aa, Artificial Sequence
  Synthetic Construct
ARDSYYYDSSGALGY

SEQ ID NO: 114 - protein, 17 aa, Artificial Sequence
  Synthetic Construct
ARPGYSSGWYDGTYFDY

SEQ ID NO: 115 - protein, 12 aa, Artificial Sequence
  Synthetic Construct
TREPGRLWAFDI

SEQ ID NO: 116 - protein, 8 aa, Artificial Sequence
  Synthetic Construct
AVFGSGSS

SEQ ID NO: 117 - protein, 8 aa, Artificial Sequence
  Synthetic Construct
AVFGSGSS

SEQ ID NO: 118 - protein, 17 aa, Artificial Sequence
  Synthetic Construct
AREGGWYGGDYYYGMDV

SEQ ID NO: 119 - protein, 15 aa, Artificial Sequence
  Synthetic Construct
AKDGDGSGPPYYFDY

SEQ ID NO: 120 - protein, 24 aa, Artificial Sequence
  Synthetic Construct
ARDRGITMVRGLIIKYYYYYGLDV

SEQ ID NO: 121 - protein, 13 aa, Artificial Sequence
  Synthetic Construct
ARDDNWNDGDFDY

SEQ ID NO: 122 - protein, 19 aa, Artificial Sequence
  Synthetic Construct
AKDFTYYYGSGNYYNWFDP

SEQ ID NO: 123 - protein, 15 aa, Artificial Sequence
  Synthetic Construct
ARTSDYDYYYYGMDV

SEQ ID NO: 124 - protein, 8 aa, Artificial Sequence
  Synthetic Construct
ARHTPGAF

SEQ ID NO: 125 - protein, 17 aa, Artificial Sequence
  Synthetic Construct
TRVLFYYYGSSYVFFDY

SEQ ID NO: 126 - protein, 6 aa, Artificial Sequence
  Synthetic Construct
QSVSSY

SEQ ID NO: 127 - protein, 6 aa, Artificial Sequence
  Synthetic Construct
QSIDTY

SEQ ID NO: 128 - protein, 6 aa, Artificial Sequence
  Synthetic Construct
QSVSNW

SEQ ID NO: 129 - protein, 6 aa, Artificial Sequence
  Synthetic Construct
QSIDTW

SEQ ID NO: 130 - protein, 6 aa, Artificial Sequence
  Synthetic Construct
QDIRNW

SEQ ID NO: 131 - protein, 6 aa, Artificial Sequence
  Synthetic Construct
QGISNS

SEQ ID NO: 132 - protein, 6 aa, Artificial Sequence
  Synthetic Construct
QGISNY

SEQ ID NO: 133 - protein, 6 aa, Artificial Sequence
  Synthetic Construct
QGISSA

SEQ ID NO: 134 - protein, 6 aa, Artificial Sequence
  Synthetic Construct
QGISSW

SEQ ID NO: 135 - protein, 6 aa, Artificial Sequence
  Synthetic Construct
QSVSSY

SEQ ID NO: 136 - protein, 6 aa, Artificial Sequence
  Synthetic Construct
QGISSY

SEQ ID NO: 137 - protein, 6 aa, Artificial Sequence
  Synthetic Construct
QSISSW

SEQ ID NO: 138 - protein, 9 aa, Artificial Sequence
  Synthetic Construct
SGINLGRYR

SEQ ID NO: 139 - protein, 11 aa, Artificial Sequence
  Synthetic Construct
QSLVHSNGDTY

SEQ ID NO: 140 - protein, 6 aa, Artificial Sequence
  Synthetic Construct
QDISNF

SEQ ID NO: 141 - protein, 3 aa, Artificial Sequence
  Synthetic Construct
DAS

SEQ ID NO: 142 - protein, 3 aa, Artificial Sequence
  Synthetic Construct
AAS

SEQ ID NO: 143 - protein, 3 aa, Artificial Sequence
  Synthetic Construct
KAS

SEQ ID NO: 144 - protein, 3 aa, Artificial Sequence
  Synthetic Construct
SAS

SEQ ID NO: 145 - protein, 3 aa, Artificial Sequence
  Synthetic Construct
AAS

SEQ ID NO: 146 - protein, 3 aa, Artificial Sequence
  Synthetic Construct
AAS

SEQ ID NO: 147 - protein, 3 aa, Artificial Sequence
  Synthetic Construct
AAS

SEQ ID NO: 148 - protein, 3 aa, Artificial Sequence
  Synthetic Construct
DAS

SEQ ID NO: 149 - protein, 3 aa, Artificial Sequence
  Synthetic Construct
AAS

SEQ ID NO: 150 - protein, 3 aa, Artificial Sequence
  Synthetic Construct
DAS

SEQ ID NO: 151 - protein, 3 aa, Artificial Sequence
  Synthetic Construct
AAS

SEQ ID NO: 152 - protein, 3 aa, Artificial Sequence
  Synthetic Construct
KAS

SEQ ID NO: 153 - protein, 7 aa, Artificial Sequence
  Synthetic Construct
YYSDSSK

SEQ ID NO: 154 - protein, 3 aa, Artificial Sequence
  Synthetic Construct
YTS

SEQ ID NO: 155 - protein, 9 aa, Artificial Sequence
  Synthetic Construct
QQRSNWPLT

SEQ ID NO: 156 - protein, 10 aa, Artificial Sequence
  Synthetic Construct
QQSYSSPGIT

SEQ ID NO: 157 - protein, 9 aa, Artificial Sequence
  Synthetic Construct
LQYVSYPLT

SEQ ID NO: 158 - protein, 9 aa, Artificial Sequence
  Synthetic Construct
QQYKTYPFT

SEQ ID NO: 159 - protein, 9 aa, Artificial Sequence
  Synthetic Construct
QQADSSPRT

SEQ ID NO: 160 - protein, 9 aa, Artificial Sequence
  Synthetic Construct
QQYKSYPYT

SEQ ID NO: 161 - protein, 9 aa, Artificial Sequence
  Synthetic Construct
QQYKTYPYT

SEQ ID NO: 162 - protein, 9 aa, Artificial Sequence
  Synthetic Construct
HQFNNYPFT

SEQ ID NO: 163 - protein, 9 aa, Artificial Sequence
  Synthetic Construct
QQYNSYPYT

SEQ ID NO: 164 - protein, 8 aa, Artificial Sequence
  Synthetic Construct
QQRSNWWT

SEQ ID NO: 165 - protein, 9 aa, Artificial Sequence
  Synthetic Construct
QQLNSYPRT

SEQ ID NO: 166 - protein, 9 aa, Artificial Sequence
  Synthetic Construct
QQYNSYSRT

SEQ ID NO: 167 - protein, 10 aa, Artificial Sequence
  Synthetic Construct
MIWHRSALFI

SEQ ID NO: 168 - protein, 9 aa, Artificial Sequence
  Synthetic Construct
SQSTHVPYT

SEQ ID NO: 169 - protein, 9 aa, Artificial Sequence
  Synthetic Construct
QQGHTLPYT

SEQ ID NO: 170 - protein, 113 aa, Artificial Sequence
  Synthetic Construct
QVQLQQSGPELVKPGASVKMSCKASGFTFTDSVISWVKQRTGQGLEWIGEIYPGSGSIYYNEKFKGKATLTADKSSNTAYMQLRSLTSEDSAVYFCAMRRSYWGQGTLVTVSA

SEQ ID NO: 171 - protein, 112 aa, Artificial Sequence
  Synthetic Construct
DVLMTQTPLSLPVSLGDQASISCRSSQSIVHSNGNTYLEWYLQKPGQSPKLLIYKVSNRFSGVPDRFSGSGSGTDFTLKISRVEAEDLGVYYCFQGSHVPLTFGAGTKLELK

SEQ ID NO: 172 - protein, 113 aa, Artificial Sequence
  Synthetic Construct
QIQLQQSGPELVKPGASVKMSCEASGFTFTDSVITWVKQRPGQGLEWIGEIYPGSGNFYYNEKFKGKATLTADKSSNTAYMQLRSLTSEDSAVYFCAMRRSSWGQGTLVTVSA

SEQ ID NO: 173 - protein, 112 aa, Artificial Sequence
  Synthetic Construct
DVLMTQTPLSLPVSLGDQASISCRSSQTIVHSNSKTYLEWYLQKPGQSPKLLIYKVSNRFSGVPDRFSGSGSGTDFTLKISRVEAEDLGVYYCFQGSHVPLTFGAGTKLELK

SEQ ID NO: 174 - protein, 125 aa, Artificial Sequence
  Synthetic Construct
QVQLQQSGGGLVQPGGSLRLSCAASGFTFSSYAMSWVRQAPGKGLEWVSAISGSGGSTYYADSVKGRFTVSRDNSKNTLYLQMNSLRAEDTAVYYCARLGYCSSTSCYLSAFDIWGQGTMVTVSS

SEQ ID NO: 175 - protein, 107 aa, Artificial Sequence
  Synthetic Construct
EIVLTQSPSTLSASVGDRVTITCRASQSISSWLAWYQQKPGKAPKLLIYDASSLESGVPSRFSGSGSGTEFTLTISSLQPDDFATYYCQQYNSYPLTFGGGTKVEIK

SEQ ID NO: 176 - protein, 120 aa, Artificial Sequence
  Synthetic Construct
QIQLVQSGAEVKKPGKSLKIACKGSGYSFSNYWIGWVRQMPGKGLEWMGIIYPGDSDTRYSPSFHGQVTISADKSISTAYLQWSSLKASDTAMYYCRVIINGTTSGFDYWGQGTLVIVSS

SEQ ID NO: 177 - protein, 107 aa, Artificial Sequence
  Synthetic Construct
ETTLTQSPATLSVSPGERATLSCRASQSVSSNLAWYQQKPGQAPRLLMYGASTRATGIPARFSGSGSGTEFTLTISSLQSEDFAVYYCQHYNNLPLTFGGGTKVDLK

SEQ ID NO: 178 - protein, 117 aa, Artificial Sequence
  Synthetic Construct
EVQLQQSGAELVKPGASVKLSCTASGFNIKDTYIHWVKQRPEQGLEWIGRIDPANGNTKYDPKFQGKATITADTSSNIVYVQFSSLTSEDTAVYYCGRSGGNYVGYWGQGTTLTVSS

SEQ ID NO: 179 - protein, 113 aa, Artificial Sequence
  Synthetic Construct
DIVMSQSPSSPTVSVGEKVTMTCKSSQSLLDSGNQKNYLAWYQQKPGQSPKLLIYWASTRKSGVPDRFTGSGSGTDFTLSISSVKAEDLAVYYCQQYYTYPWTFGGGTKLEIK

SEQ ID NO: 180 - protein, 117 aa, Artificial Sequence
  Synthetic Construct
EVQLQQSGAELVKPGASVKLSCTASGFNIKDTYMHWVKERPEQGLEWIGRIDPANGNTKYDPKFQGKATITADTSSNTAYLQLSSLTSEDTAVYYCGRSRGNYFDYWGQGTTLTVSS

SEQ ID NO: 181 - protein, 111 aa, Artificial Sequence
  Synthetic Construct
DIVMSQPPSSLAVSVGEKVTMTCKSSQSLKSNQKNYLAWYQQKPGQSPKLLIYWASTRESGVPDRFTGSGSGTDFTLTISSVKAEDLAVYYCQQYYTYPWTFGGGTKLEIK

SEQ ID NO: 182 - protein, 113 aa, Artificial Sequence
  Synthetic Construct
QVQLVQSGAEVKKPGTSVKVSCKASGYTFTTYYMHWVRQAPGQGLEWMGLINPSAGNTRNAQKFQGRVTMTRDTSTNTVYMELSSLRSEDTAVYYCARELDIWGQGTKVTVSS

SEQ ID NO: 183 - protein, 107 aa, Artificial Sequence
  Synthetic Construct
AIQMTQSPSSLSASVGDRVTITCRASQDIRNDLGWYQQKPGKAPKLLIYAASSLQSGVPSRFSGNGSGTDFTLTINSLQPEDFATYYCLQDFNFPFTFGPGTTVDIN

SEQ ID NO: 184 - protein, 120 aa, Artificial Sequence
  Synthetic Construct
QVQLVESGGGVVQSGRSLRLSCAASGFTFSSYGMHWVRQAPGKGLEWVAVIWYDGSNKYYADSVKDRFTISRDNSKKTVYLQMNSLRAEDTAVYYCAREGMVRGALFDYWGQGTLVTVSS

SEQ ID NO: 185 - protein, 108 aa, Artificial Sequence
  Synthetic Construct
EIVMTQSPATLSLSPGERATLSCRASQSVSSSYLSWYQQKPGQAPRLLIYGASTRATGIPARFSGSGSGPDLTLTISSLQPEDFAVYYCQQDYNLPYTFGQGTKLEIK

SEQ ID NO: 186 - protein, 119 aa, Artificial Sequence
  Synthetic Construct
EVQLVQSGAEVKKPGESLKISCKGSGYSFTSYWIGWVRQMPGKGLEWMGVIYPGDSDTRYSPSFQGQVTMSADKSISTAYLQWSSLKASDSAMYYCARQLRDYYGMDVWGQGTTVTVSS

SEQ ID NO: 187 - protein, 108 aa, Artificial Sequence
  Synthetic Construct
EIVMTQSPATLSLSPGERATLSCRASQTISSNYFSWYQQKPGQAPRLLIYGASTRATGIPARFSGSGSETDFTLTISSLQPEDFAVYYCQQDYNLPRTFGQGTKVEIK

SEQ ID NO: 188 - protein, 119 aa, Artificial Sequence
  Synthetic Construct
EVQLVQSGAEVKKPGESLKISCKGSGYSFTSYWIGWVRQMPGKGLEWMGIIYPGDSDTRYSPSFQGQVTISADKSISTAYLHWSSLKASDTAMYYCARQLRDYYSMDVWGQGTTVTVSS

SEQ ID NO: 189 - protein, 108 aa, Artificial Sequence
  Synthetic Construct
EIVMTQSPATLSLSPGERATLSCRASQSVSSSYLSWYQQKPGQAPRLLIYGASTRATGIAARFSGSGSGTDFTLTISSLQPEDFAVYYCQQDYNLPRTFGQGTKVEIK

SEQ ID NO: 190 - protein, 114 aa, Artificial Sequence
  Synthetic Construct
EVQLQQSGPELVKPGASVKMSCKASGYTFTSYNIHWVKQKPGQGLEWIGYINPYNDGTKYSEKFKGKATLTSDRSSSTAYMEVSSLTSEDSAVYYCAIYGNSYWGQGSTLTVSS

SEQ ID NO: 191 - protein, 112 aa, Artificial Sequence
  Synthetic Construct
DIVMTQAAPSIPVTPGESVSISCRSSKSLLHSNGNTYLYWFLQRPGQSPQRLIYYMSNLDSGVPDRFSGRGSGTDFTLRISRVEAEDVGVYYCMQGLEYPYTFGGGTKLEIK

SEQ ID NO: 192 - protein, 118 aa, Artificial Sequence
  Synthetic Construct
DVMLVESGGDLVKPGGSLKLSCAASGFTFSSYTMSWVRQTPEKRLEWVASISSGGGNTYYPDSVKGRFTISRDNAKNNLYLQMSSLRSEDTALYYCARFDYGSSLDSWGQGTTLTVSS

SEQ ID NO: 193 - protein, 107 aa, Artificial Sequence
  Synthetic Construct
DIVLTQSPATLSVTPGDSVSLSCRASQSISNNLHWYQQKSHESPRLLIKYASQSISGIPSRFSGSGSGTDFTLSINSVETEDFGMYFCQQSKNWPRTFGGGTKLEIK

SEQ ID NO: 194 - protein, 118 aa, Artificial Sequence
  Synthetic Construct
EVMLVESGGGLVKPGGSLKLSCAASGFTFSSYTMSWVRQTPEKRLEWVATISSGGDNTYYPDSVKGRFTISRDNAKNNLYLQMSSLRSEDTALYYCARFDYGSSLDCWGQGTTLTVSS

SEQ ID NO: 195 - protein, 107 aa, Artificial Sequence
  Synthetic Construct
DIVLTQSPATLSVTPGDSVSLSCRASQSISNYLHWYQQKSHESPRLLIKYASQSISGIPSRFSGSGSGTDFTLSINSVETEDFGMYFCQQSKSWPRTFGGGTELEIK

SEQ ID NO: 196 - protein, 120 aa, Artificial Sequence
  Synthetic Construct
EVQLVQSGAEVKKPGESLKISCKGSGYSFTSYWIGWVRQMPGKGLEWMGIIYPGDSDTRYSPSFQGQVTISADKSISTAYLQWSSLKASDTAMYYCARRGYRSSWYFDYWGQGTLVTVSS

SEQ ID NO: 197 - protein, 107 aa, Artificial Sequence
  Synthetic Construct
AIQMTQSPSSLSASVGDRVTITCRASQGIRNDLGWYQQKPGKAPKLLIYAASSLQSGVPSRFSGSGSGTDFTFTISSLQPEDFATYYCLQDYNYPLTFGGGTKVEIK

SEQ ID NO: 198 - protein, 118 aa, Artificial Sequence
  Synthetic Construct
EVQLVESGGGVVRPGGSLRLSCAASGFTFDDYGMSWVRQAPGKGLEWVSGINWNGGSTGYADSVKGRFTISRDNAKNSLYLQMNSLRAEDTALYHCAREGGELLMDYWGQGTLVTVSS

SEQ ID NO: 199 - protein, 105 aa, Artificial Sequence
  Synthetic Construct
EIVLTQSPATLSLSPGERATLSCRASQSVSTYLAWYQQKPGQAPRLLIYDNRATGIPPRFSGSGSGTDFTLTISSLEPEDFAVYYCQQRSNWPPTFGGGTTVEIK

SEQ ID NO: 200 - protein, 125 aa, Artificial Sequence
  Synthetic Construct
EVQLLESGGGLVQPGGSLRLSCAASGFTFSHYSMVWVRQAPGKGLEWVSYIYPSGGTSYADSVKGRFTISRDNSKNTLYLQMNSLRAEDTAVYYCARHWRGYSSSWYHPAYFDYWGQGTLVTVSS

SEQ ID NO: 201 - protein, 105 aa, Artificial Sequence
  Synthetic Construct
DIQMTQSPATLSLSPGERATLSCRASQSVSSYLAWYQQKPGQAPRLLIYDNRATGIPARFSGSGSGTDFTLTISSLEPEDFAVYYCQQRSNWPLTFGGGTKVEIK

SEQ ID NO: 202 - protein, 126 aa, Artificial Sequence
  Synthetic Construct
EVQLLESGGGLVQPGGSLRLSCAASGFTFSWYPMMWVRQAPGKGLEWVSSIYPSGGTTTYADSVKGRFTISRDNSKNTLYLQMNSLRAEDTAVYYCARSYYYDSSGYYSHDAFDIWGQGTMVTVSS

SEQ ID NO: 203 - protein, 108 aa, Artificial Sequence
  Synthetic Construct
DIQMTQSPSSLSASVGDRVAITCRASQSIDTYLNWYQQKPGKAPKLLIYAASKLEDGVPSRFSGSGTGTDFTLTIRSLQPEDFASYFCQQSYSSPGITFGPGTKVEIK

SEQ ID NO: 204 - protein, 122 aa, Artificial Sequence
  Synthetic Construct
EVQLLESGGGLVQPGGSLRLSCAASGFTFSDYEMHWVRQAPGKGLEWVSSIWPSGGLTKYADPVKGRFTISRDNSKNTLYLQMNSLRAEDTAVYYCARDSYYYDSSGALGYWGQGTLVTVSS

SEQ ID NO: 205 - protein, 107 aa, Artificial Sequence
  Synthetic Construct
DIQMTQSPSTLSASVGDRVTITCRASQSVSNWLAWYQQKPGKAPKLLIYKASSLESGVPSRFSGSGSGTEFTLTISSLQPDDFATYYCLQYVSYPLTFGGGTKVDIK

SEQ ID NO: 206 - protein, 124 aa, Artificial Sequence
  Synthetic Construct
EVQLLESGGGLVQPGGSLRLSCAASGFTFSYYDMYWVRQAPGKGLEWVSRIYSSGGHTWYADSVKGRFTISRDNSKNTLYLQMNSLRAEDTAVYYCARPGYSSGWYDGTYFDYWGQGTLVTVSS

SEQ ID NO: 207 - protein, 107 aa, Artificial Sequence
  Synthetic Construct
DIQMTQSPSTLSASVGDRVTITCRASQSIDTWLAWYRQKPGKAPNVVIHSASTLQSGVPARFSGSGFGTEWTLTITNLQPDDFATYYCQQYKTYPFTFGQGTKLEIK

SEQ ID NO: 208 - protein, 119 aa, Artificial Sequence
  Synthetic Construct
EVQLLESGGGLVQPGGSLRLSCAASGFTFSHYQMEWVRQAPGKGLEWVSSISPSGGFTSYADSVKGRFTISRDNSKNTLYLQMNSLRAEDTAVYYCTREPGRLWAFDIWGQGTMVTVSS

SEQ ID NO: 209 - protein, 107 aa, Artificial Sequence
  Synthetic Construct
DIQMTQSPSFVSASVGDRVTITCRASQDIRNWLAWYQQESGKAPRLLISAASSRHSGVSSRFSGSGSGTDFTLTITSLQPEDSATYFCQQADSSPRTFGQGTKVEIK

SEQ ID NO: 210 - protein, 115 aa, Artificial Sequence
  Synthetic Construct
QVQLVQSGAEVKKPGASVKVSCKASGYTFTGYYMHWVRQAPGQGLEWMGWINPNSGGTNYAQKFQGRVTMTRDTSINTAYMELSRLRSDDTAVYYCAVFGSGSSWGQGTLVTVSS

SEQ ID NO: 211 - protein, 107 aa, Artificial Sequence
  Synthetic Construct
DIQMTQSPSSLSASVGDRVTITCRASQGISNSLAWFQQKPGKAPKSLIYAASSLQSGVPSKFSGSGSGTDFTLTISSLQPEDFATYYCQQYKSYPYTFGQGTKLEIK

SEQ ID NO: 212 - protein, 115 aa, Artificial Sequence
  Synthetic Construct
QVQLVQSGAEVKKPGASVKVSCKASGNTFTGYYIHWVRQAPGQGLEWMGWIKPSTGDTNYAQNFLDRVTMTRDTSISTAYMELSRLRSDDTAVYYCAVFGSGSSWGQGTLVTVSS

SEQ ID NO: 213 - protein, 107 aa, Artificial Sequence
  Synthetic Construct
DIHMTQSPSSLSAFVGDRVTITCRASQGISNYLAWFQQKPGKAPKSLIYAASSLQSGVPSKFSGSGSGTDFTLTINNLQPEDFATYYCQQYKTYPYTFGQGTKLEIK

SEQ ID NO: 214 - protein, 124 aa, Artificial Sequence
  Synthetic Construct
QVQLVESGGGVVQPGRSLRLSCAASGFTFSSYGMHWVRQAPGKGLEWVAVIWYDGSNKYYADSVKGRFTISRDNSKNTLYLQMNSLRAEDAAVYYCAREGGWYGGDYYYGMDVWGQGTTVTVSS

SEQ ID NO: 215 - protein, 105 aa, Artificial Sequence
  Synthetic Construct
AIQLTQSPSSLSASVGDRVTITCRASQGISSAWYQQKPGKAPKLLIYDASSLESGVPSRFSGSGSGTDFTLTISSLQPEDFATYYCHQFNNYPFTFGPGTKVDIK

SEQ ID NO: 216 - protein, 122 aa, Artificial Sequence
  Synthetic Construct
EVQLLESGGGLVQPGGSLRLSCVASGFTFSSYAMSWVRQAPGKGLEWVSGISGRGGSPNYADSVKGRFTISRDNSKNTLYLQMNSLRAEDTAVYYCAKDGDGSGPPYYFDYWGQGTLVTVSS

SEQ ID NO: 217 - protein, 107 aa, Artificial Sequence
  Synthetic Construct
DIQMTQSPSSLSASVGDRVTITCRASQGISSWLAWYQQKPEKAPKSLIYAASSLQSGVPSRFSGSGSGTDFTLTISSLQPEDFATYYCQQYNSYPYTFGQGTKLEIK

SEQ ID NO: 218 - protein, 131 aa, Artificial Sequence
  Synthetic Construct
QVQLMESGGGVVQPGRSLRLSCAASGFTFSGYGMHWVRQAPGKGLEWVAVIWSDGSNRYYTDSVKGRFTISRDNSKNTLSLQMNSLRAEDTAVYYCARDRGITMVRGLIIKYYYYYGLDVWGQGTSVTVSS

SEQ ID NO: 219 - protein, 104 aa, Artificial Sequence
  Synthetic Construct
EIVLTQSPATLSLSPGERATLSCRASQSVSSYLAWYQQKPGQAPRLLIYDNRATGIPARFSGSGSGTDFTLTISSLEPEDFAVYYCQQRSNWWTFGQGTKVEIK

SEQ ID NO: 220 - protein, 120 aa, Artificial Sequence
  Synthetic Construct
QVQLVESGGGVVQPGRSLRLSCAASGFTFSSFGMHWVRQAPGKGLEWVAVIYYDGSNKYYADSVKGRFTISRDNSKNTLYLQMNSLRAEDTAVYYCARDDNWNDGDFDYWGQGTLVTVSS

SEQ ID NO: 221 - protein, 107 aa, Artificial Sequence
  Synthetic Construct
DIQLTQSPSFLSASVGDRVTITCRASQGISSYLAWYQQKPGKAPKLLIYAASTLQSGVPSRFSGSGSGTEFTLTISSLQPEDFATYYCQQLNSYPRTFGQGTKVEIK

SEQ ID NO: 222 - protein, 126 aa, Artificial Sequence
  Synthetic Construct
EVQLLESGGGLVQPGESLRLSCAASGFTFNRFVMSWVRQAPGKGLEWVSTISGSGGSTYYADSVKGRFTISRDNSKNTLYLQMNSLRAEDTAVYYCAKDFTYYYGSGNYYNWFDPRGQGTLVTVSS

SEQ ID NO: 223 - protein, 107 aa, Artificial Sequence
  Synthetic Construct
DIQMTQSPSTLSTSVGDRVTITCRASQSISSWLAWYQQKPGKAPKLLIYKASSLESGVPSRFSGSGSGTEFTLTISSLQPDDFATYYCQQYNSYSRTFGQGTKVEIK

SEQ ID NO: 224 - protein, 121 aa, Artificial Sequence
  Synthetic Construct
QVQLQQWGAGLLKPSETLSLTCAVYGGSFSGYYWSWIRQPPGKGLEWIGEINHSGGTNYNPSLKSRVTISVDTSKNHFSLKLSSVTAADTAVYYCARTSDYDYYYYGMDVWGQGTTVTVSS

SEQ ID NO: 225 - protein, 114 aa, Artificial Sequence
  Synthetic Construct
QPVLTQPTSLSDGASARLTCTLRSGINLGRYRIFWYQQKPESPPRYLLSYYSDSSKHQGSGVPSRFSGSKDASSNAGILVISGLQSEDEADYYCMIWHRSALFIFGSGTKVTVL

SEQ ID NO: 226 - protein, 115 aa, Artificial Sequence
  Synthetic Construct
QVQLQQSGPELVKPGASVKLSCKASGYTFTSYEINWLKQRPGQGLEWIGLIYPRDGDTKYNEKFKGKATLTADTSSSTAYMELHSLTSEDSAVYFCARHTPGAFWGQGTLVTVSA

SEQ ID NO: 227 - protein, 112 aa, Artificial Sequence
  Synthetic Construct
DVVMTQTPLSLPVSLGDQASISCRSSQSLVHSNGDTYLHWYLQKPGQSPKLLIYKVSNRFSGVPDRFSGSGSGTDFTLKISRVEAEDLEIYFCSQSTHVPYTFGGGTKLEIK

SEQ ID NO: 228 - protein, 124 aa, Artificial Sequence
  Synthetic Construct
DVKLVESGEGLVKPGGSLKLSCAASGFTFSRYAMSWVRQTPEKRLEWVAYISSGGDYIHYGETVKGRFTISRDNARNTLYLQMSSLKSEDTAMYYCTRVLFYYYGSSYVFFDYWGQGTTLTVSS

SEQ ID NO: 229 - protein, 107 aa, Artificial Sequence
  Synthetic Construct
DIQMTQTTSSLSVSLGDRVTISCRASQDISNFLNWYQQKPDGTVNLLIYYTSKLHSGVPSRFSGGGSGRDYSLTINNLEQEDIASYFCQQGHTLPYTFGGGTKLEIK

SEQ ID NO: 230 - DNA, 339 bp, Artificial Sequence
  Synthetic Construct
caggtgcagctgcagcagagcggtcccgagctggtgaaacctggcgcatcagtcaaaatgagctgcaaggcctccggcttcacttttaccgactcagtgatcagctgggtcaagcagcgaaccggtcagggactggagtggatcggagaaatctaccctggatctgggagtatctactataacgagaagttcaaagggaaggcaacactgactgccgacaaaagctccaatacagcctatatgcagctgcgatccctgacttctgaagatagcgccgtgtacttttgcgcaatgcggaggtcctattggggtcagggcaccctggtgacagtctctgct

SEQ ID NO: 231 - DNA, 336 bp, Artificial Sequence
  Synthetic Construct
gacgtgctgatgacccagacacccctgagtctgcctgtctcactgggagatcaggcttctatcagttgccgaagctcccagagcatcgtgcattccaacggaaatacctacctggagtggtatctgcagaagccagggcagtcccccaagctgctgatctacaaagtgtctaaccggttcagtggcgtcccagacaggttttcaggtagcggctccggaactgatttcaccctgaaaatttcccgggtggaggcagaagacctgggtgtctactattgcttccagggcagccatgtgcccctgacttttggggccggtaccaagctggagctgaaa

SEQ ID NO: 232 - DNA, 339 bp, Artificial Sequence
  Synthetic Construct
cagatccagctgcagcagtccggtcccgagctggtgaaacctggcgcatctgtcaagatgagttgcgaagcctcaggcttcacttttaccgactccgtgattacctgggtcaaacagcgcccaggccagggactggagtggatcggagaaatctaccccggatctgggaacttctactataatgagaagtttaaagggaaggcaacactgactgccgacaagagctccaacaccgcctacatgcagctgcgatcactgacaagcgaagatagcgccgtgtacttctgcgcaatgcggaggtctagttggggtcagggcaccctggtgacagtctctgct

SEQ ID NO: 233 - DNA, 336 bp, Artificial Sequence
  Synthetic Construct
gacgtgctgatgacccagacacccctgtctctgcctgtcagtctgggagatcaggcttctatcagttgccgaagctcccagaccatcgtgcattcaaacagcaagacatacctggagtggtatctgcagaaaccaggccagtcccccaagctgctgatctacaaagtgtcaaatcggttctctggagtcccagacaggttttccggttctggcagtggaactgatttcaccctgaagatttctcgggtggaggcagaagacctgggtgtctactattgcttccaggggagccatgtgcccctgacttttggggccggtaccaagctggagctgaaa

SEQ ID NO: 234 - DNA, 375 bp, Artificial Sequence
  Synthetic Construct
caggtgcagctgcagcagtcggggggaggcttggtacagcctggggggtccctgagactctcctgtgcagcctctggattcacctttagcagctatgccatgagctgggtccgccaggctccagggaaggggctggagtgggtctcagctattagtggtagtggtggtagcacatactacgcagactccgtgaagggccggttcaccgtctccagagacaattccaagaacacgctgtatctgcaaatgaacagcctgagagccgaggacacggccgtatattactgtgcgaggctaggatattgtagtagtaccagctgctatttgtctgcttttgatatctggggccaagggacaatggtcaccgtctcttca

SEQ ID NO: 235 - DNA, 321 bp, Artificial Sequence
  Synthetic Construct
gaaattgtgttgacacagtctccttccaccctgtctgcatctgtaggagacagagtcaccatcacttgccgggccagtcagagtattagtagctggttggcctggtatcagcagaaaccagggaaagcccctaagctcctgatctatgatgcctccagtttggaaagtggggtcccatcaaggttcagcggcagtggatctgggacagaattcactctcaccatcagcagcctgcagcctgatgattttgcaacttattactgccaacagtataatagttacccgctcactttcggcggagggaccaaggtggagatcaaa

SEQ ID NO: 236 - DNA, 366 bp, Artificial Sequence
  Synthetic Construct
cagatccagctggtgcagtctggcgccgaagtgaagaagcctggcaagagcctgaagatcgcctgcaagggctccggctacagcttcagcaactactggatcggctgggtgcgccagatgcctggaaaaggactggaatggatgggcattatctaccctggcgacagcgacacccggtacagccccagcttccacggccaggtgacaatcagcgccgacaagagcatctccaccgcctacctgcagtggtcctccctgaaggccagcgacaccgccatgtactattgtgccagaggcgtgatcatcaacggcaccaccagcggcttcgactattggggacagggcaccctggtgatcgtgtcctcc

SEQ ID NO: 237 - DNA, 321 bp, Artificial Sequence
  Synthetic Construct
gagacaaccctgacccagagccccgccaccctgtccgtgtctccaggcgagagagccaccctgagctgcagagccagccagagcgtgtccagcaacctggcctggtatcagcagaagcccggccaggcccccagactgctgatgtacggcgccagcaccagagccaccggcatccctgccagattcagcggcagcggctccggcaccgagttcaccctgaccatcagcagcctgcagagcgaggacttcgccgtgtactactgccagcactacaacaacctgcccctgaccttcggcggaggcaccaaggtggacctgaag

SEQ ID NO: 238 - DNA, 351 bp, Artificial Sequence
  Synthetic Construct
gaagtccaactccaacagtctggggcagaacttgtcaaacctggggcttcagtaaaattgagttgcacagcaagtggctttaacatcaaagacacatatattcattgggtgaagcaacgaccagaacaaggcttggagtggatcggtaggattgaccctgcaaacgggaatacaaaatatgaccctaaattccagggaaaggctacaataacagcagacaccagcagtaacattgtctatgtgcaatttagctctcttacctctgaggacactgctgtctattattgcggacgtagtggcgggaattatgtgggttattggggccaggggacaacactcaccgtatcctct

SEQ ID NO: 239 - DNA, 339 bp, Artificial Sequence
  Synthetic Construct
gatatagtaatgtcccagtctccttcatcacctactgtgtcagttggagaaaaagtcaccatgacctgtaagtcctcacagtccctcttggacagcgggaatcagaaaaattatctcgcatggtatcagcaaaagccagggcagtcccctaagctgttgatctattgggcaagtacaaggaaaagtggcgtgcctgatagattcacagggagcggcagcgggacagacttcactttgagcatctcttcagtaaaagccgaagacctggcagtgtactactgtcagcaatattatacctacccttggacttttggtggcgggaccaaactggaaataaaa

SEQ ID NO: 240 - DNA, 351 bp, Artificial Sequence
  Synthetic Construct
gaggttcaacttcagcaatcaggggctgagcttgtaaaacctggagcctctgtaaaactctcttgtaccgcctccgggttcaacataaaagatacatatatgcactgggtaaaggagcggcccgaacagggactcgaatggatcgggaggattgacccagctaacggaaataccaagtatgatccaaaatttcaggggaaagctacaataaccgccgatacttctagtaatacagcatatcttcagctcagcagcttgacaagcgaagataccgcagtttactactgcggtcgatcccgagggaattattttgactactggggccagggtactactctcacagtaagtagc

SEQ ID NO: 241 - DNA, 339 bp, Artificial Sequence
  Synthetic Construct
gacatagtaatgagccagccacctagttcacttgccgtaagtgtgggtgaaaaggtgactatgacctgtaaaagtagtcagagcctcctttactcatcaaatcagaagaattacttggcctggtatcaacagaaacctggacaaagccccaaactcctcatatactgggcctctacccgagagtccggcgtaccagatcggtttaccggttctggatcaggtacagactttacacttaccatctcttcagtgaaggctgaggacttggccgtgtattattgtcaacaatattatacatatccttggacttttggcggagggacaaagctcgaaataaag

SEQ ID NO: 242 - DNA, 339 bp, Artificial Sequence
  Synthetic Construct
caggtgcagctggtgcagtctggcgccgaagtgaagaaacccggcacctccgtgaaggtgtcctgcaaggcttccggctacacctttaccacctactacatgcactgggtgcgacaggcccctggacagggcctggaatggatgggcctgatcaacccttccgccggcaacaccagaaacgcccagaaattccagggcagagtgaccatgacccgggacacctccaccaacaccgtgtacatggaactgtcctccctgcggagcgaggacaccgccgtgtactactgtgccagagagctggacatctggggccagggcaccaaagtgaccgtgtcctct

SEQ ID NO: 243 - DNA, 321 bp, Artificial Sequence
  Synthetic Construct
gccatccagatgacccagtcccccagctccctgtctgcctctgtgggcgacagagtgaccatcacctgtcgggcctctcaggacatccggaacgacctgggctggtatcagcagaagcctggcaaggcccccaagctgctgatctacgccgcttccagtctccagtccggcgtgccctccagattctccggcaatggctctggcaccgacttcaccctgaccatcaactccctccagcccgaggacttcgccacctactactgtctccaagacttcaacttccccttcaccttcggccctggcaccaccgtggacatcaac

SEQ ID NO: 244 - DNA, 360 bp, Artificial Sequence
  Synthetic Construct
caggtgcagctggtggagtctgggggaggcgtggtccagtctgggaggtccctgagactctcctgtgcagcgtctggattcaccttcagtagttatggcatgcactgggtccgccaggctccaggcaaggggctggagtgggtggcagttatatggtatgatggaagtaataaatactatgcagactccgtgaaggaccgattcaccatctccagagacaattccaagaaaacggtgtatctgcaaatgaacagtctgagagccgaggacacggctgtttattactgtgcgagagaagggatggttcggggagccctctttgactactggggtcagggaaccctggtcaccgtctcctca

SEQ ID NO: 245 - DNA, 324 bp, Artificial Sequence
  Synthetic Construct
gaaattgtaatgacacagtctccagccaccctgtctttgtctccaggggaaagagccaccctctcctgcagggccagtcagagtgttagcagcagctacttatcctggtaccaacagaaacctgggcaggctcccaggctcctcatctatggtgcatccaccagggccactggcatcccagccaggttcagtggcagtgggtctgggccagacctcactctcaccatcagcagcctgcagcctgaagattttgcagtttattactgtcagcaggattataacttaccgtacacttttggccaggggaccaagctggagatcaaa

SEQ ID NO: 246 - DNA, 357 bp, Artificial Sequence
  Synthetic Construct
gaggtgcagctggtgcagtctggagcagaggtgaaaaagcccggggagtctctgaagatctcctgtaagggttctggatacagttttactagttactggatcggctgggtgcgccagatgcccgggaaaggcctggagtggatgggagtcatctatcctggtgactctgataccagatatagcccgtccttccaaggccaggtcaccatgtcagccgacaagtccatcagtaccgcctacctgcagtggagcagcctgaaggcctcggacagcgccatgtattactgtgcgagacagctacgagactactacggtatggacgtctggggccaagggaccacggtcaccgtctcctca

SEQ ID NO: 247 - DNA, 324 bp, Artificial Sequence
  Synthetic Construct
gaaattgtaatgacacagtctccagccaccctgtctttgtctccaggggaaagagccaccctctcctgcagggccagtcagactatcagcagcaactacttttcctggtaccagcagaaacctgggcaggctcccaggctcctcatctatggtgcatccaccagggccactggcattccagccaggttcagtggcagtgggtctgagacagacttcactctcaccatcagcagcctgcagcctgaagattttgcagtttattactgtcagcaggattataacttacctcggacgttcggccaagggaccaaggtggaaatcaaa

SEQ ID NO: 248 - DNA, 357 bp, Artificial Sequence
  Synthetic Construct
gaggtgcagctggtgcagtctggagcagaggtgaaaaagcccggggagtctctgaagatctcctgtaagggttctggatacagctttaccagctactggatcggctgggtgcgccagatgcccgggaaaggcctggagtggatggggatcatctatcctggtgactctgataccagatacagcccgtccttccaaggccaggtcaccatctcagccgacaagtccatcagcaccgcctacctgcactggagcagcctgaaggcctcggacaccgccatgtattactgtgcgagacagctacgagactactacagtatggacgtctggggccaagggaccacggtcaccgtctcctca

SEQ ID NO: 249 - DNA, 324 bp, Artificial Sequence
  Synthetic Construct
gaaattgtaatgacacagtctccagccaccctgtctttgtctccaggggaaagagccaccctctcctgcagggccagtcagagtgttagcagcagctacttatcctggtaccagcagaaacctgggcaggctcccaggctcctcatctatggtgcatccaccagggccactggcattgcagccaggttcagtggcagtgggtctgggacagacttcactctcaccatcagcagcctgcagcctgaagattttgcagtttattactgtcagcaggattataacttacctcggacgttcggccaagggaccaaggtggaaatcaaa

SEQ ID NO: 250 - DNA, 342 bp, Artificial Sequence
  Synthetic Construct
gaggtgcagctgcagcagagcggccctgagctggtgaaacctggcgccagcgtgaagatgagctgcaaggccagcggctacaccttcaccagctacaacatccactgggtgaaacagaagcccggccagggcctggaatggattggctacatcaacccctacaacgacggcaccaagtacagcgagaagttcaagggcaaggccaccctgaccagcgacagaagcagcagcaccgcctacatggaagtgtccagcctgacctccgaggacagcgccgtgtactactgcgccatctacggcaacagctactggggccagggcagcaccctgaccgtgtccagc

SEQ ID NO: 251 - DNA, 336 bp, Artificial Sequence
  Synthetic Construct
gacatcgtgatgacccaggctgcccccagcatccccgtgacacctggcgagtccgtgtccatcagctgcagaagcagcaagagcctgctgcacagcaacggcaatacctacctgtactggttcctgcagcggcctggccagtccccccagcggctgatctactacatgagcaacctggacagcggcgtgcccgaccggtttagcggcagaggcagcggcacagactttaccctgcggatcagccgggtggaagccgaggacgtgggcgtgtactattgcatgcagggcctggaatacccctacacctttggaggcggcaccaagctggaaatcaag

SEQ ID NO: 252 - DNA, 354 bp, Artificial Sequence
  Synthetic Construct
gacgtgatgctggtcgagagcggcggagatctggtcaaacccgggggttctctgaagctgagttgtgccgcttcaggcttcactttttctagttacaccatgagctgggtgcgacagaccccagagaagcggctggaatgggtcgctagcatctcaagcggcggagggaacacctactatcccgactctgtgaaaggcagattcacaattagtcgcgataatgcaaagaacaatctgtacctgcagatgtcctctctgaggtccgaagatactgccctgtactattgtgctagatttgactatggaagttcactggattcttggggacaggggaccacactgacagtgagctcc

SEQ ID NO: 253 - DNA, 321 bp, Artificial Sequence
  Synthetic Construct
gacatcgtcctgacccagagtcctgccaccctgtctgtgacaccaggcgattctgtcagtctgtcatgtagagctagccagtccatctctaacaatctgcactggtaccagcagaagtcacatgaaagccccagactgctgatcaagtatgccagtcagtcaatcagcggtattccttcccgcttctccggctctggaagtgggacagactttactctgtccatcaactctgtggagacagaagatttcggcatgtatttttgtcagcagagcaagaattggcccaggacatttggcggagggactaagctggagatcaag

SEQ ID NO: 254 - DNA, 354 bp, Artificial Sequence
  Synthetic Construct
gaagtgatgctggtcgaaagtggaggaggactggtgaaaccaggtggaagcctgaagctgtcctgtgccgcttctggcttcactttttcaagctataccatgagctgggtgcgacagacacctgagaagcggctggaatgggtcgctacaatctcctctggaggggacaacacttactatccagatagcgtgaaaggcagattcactatttcccgcgacaatgcaaagaacaatctgtacctgcagatgagttcactgaggagcgaggataccgccctgtactattgcgctagatttgactatggaagctccctggattgttggggacaggggaccacactgaccgtgtctagt

SEQ ID NO: 255 - DNA, 321 bp, Artificial Sequence
  Synthetic Construct
gacatcgtcctgactcagagccctgccaccctgtccgtgacaccaggcgattcagtcagcctgtcctgtagagcttctcagagtatctcaaactacctgcactggtatcagcagaagagtcatgaatcacccagactgctgatcaagtacgccagccagtccatctctgggattcctagccgcttcagtggctcaggaagcgggacagactttactctgagcatcaattccgtggagacagaagatttcggcatgtatttttgtcagcagtccaagtcttggcccaggacatttggcggagggactgagctggagatcaag

SEQ ID NO: 256 - DNA, 360 bp, Artificial Sequence
  Synthetic Construct
gaggtgcaactggtgcagtctggagcagaggtgaaaaagcccggggagtctctgaagatctcctgtaagggttctggatacagctttaccagctactggatcggctgggtgcgccagatgcccgggaaaggcctggagtggatggggatcatctatcctggtgactctgataccagatacagcccgtccttccaaggccaggtcaccatctcagccgacaagtccatcagcaccgcctacctgcagtggagcagcctgaaggcctcggacaccgccatgtattactgtgcgagacgcgggtatcgcagcagctggtactttgactactggggccagggaaccctggtcaccgtctcctca

SEQ ID NO: 257 - DNA, 321 bp, Artificial Sequence
  Synthetic Construct
gccatccagatgacccagtctccatcctccctgtctgcatctgtaggagacagagtcaccatcacttgccgggcaagtcagggcattagaaatgatttaggctggtatcagcagaaaccagggaaagcccctaagctcctgatctatgctgcatccagtttacaaagtggggtcccatcaaggttcagcggcagtggatcaggcacagatttcactttcaccatcagcagcctgcagcctgaagattttgcaacttattactgtctacaagattacaattacccgctcactttcggcggagggaccaaggtggagatcaaa

SEQ ID NO: 258 - DNA, 354 bp, Artificial Sequence
  Synthetic Construct
gaggtgcagctggtggagtctgggggaggtgtggtacggccgggggggtccctgagactctcctgtgcagcctctggattcacctttgatgattatggcatgagctgggtccgccaagctccagggaaggggctggagtgggtctctggtattaattggaatggtggtagcacaggttatgcagactctgtgaagggccgattcaccatctccagagacaacgccaagaactccctgtatctgcaaatgaacagtctgagagccgaggacacggccttgtatcactgtgcgagagaagggggggagctattaatggactattggggccagggaaccctggtcaccgtctcctca

SEQ ID NO: 259 - DNA, 321 bp, Artificial Sequence
  Synthetic Construct
gaaattgtgttgacacagtctccagccaccctgtctttgtctccaggggaaagagccaccctctcctgcagggccagtcagagtgttagcacctacttagcctggtaccaacagaaacctggccaggctcccaggctcctcatctatgatgcatccaacagggccactggcatcccacccaggttcagtggcagtgggtctgggacagacttcactctcaccatcagcagcctagagcctgaagattttgcagtttattactgtcagcagcgtagcaactggcctcctactttcggcggagggaccacggtggagatcaaa

SEQ ID NO: 260 - DNA, 375 bp, Artificial Sequence
  Synthetic Construct
gaagttcaattgttagagtctggtggcggtcttgttcagcctggtggttctttacgtctttcttgcgctgcttccggattcactttctctcattactctatggtttgggttcgccaagctcctggtaaaggtttggagtgggtttcttatatctatccttctggtggcacttcgtatgctgactccgttaaaggtcgcttcactatctctagagacaactctaagaatactctctacttgcagatgaacagcttaagggctgaggacacggccgtgtattactgtgcgagacattggcgggggtatagcagcagctggtaccacccggcgtactttgactactggggccagggcaccctggtcaccgtctcaagc

SEQ ID NO: 261 - DNA, 321 bp, Artificial Sequence
  Synthetic Construct
gacatccagatgacccagtctccagccaccctgtctttgtctccaggggaaagagccaccctctcctgcagggccagtcagagtgttagcagctacttagcctggtaccaacagaaacctggccaggctcccaggctcctcatctatgatgcatccaacagggccactggcatcccagccaggttcagtggcagtgggtctgggacagacttcactctcaccatcagcagcctagagcctgaagattttgcagtttattactgtcagcagcgtagcaactggcctctcactttcggcggagggaccaaggtggagatcaaa

SEQ ID NO: 262 - DNA, 378 bp, Artificial Sequence
  Synthetic Construct
gaagttcaattgttagagtctggtggcggtcttgttcagcctggtggttctttacgtctttcttgcgctgcttccggattcactttctcttggtaccctatgatgtgggttcgccaagctcctggtaaaggtttggagtgggtttcttctatctatccttctggtggcactactacttatgctgactccgttaaaggtcgcttcactatctctagagacaactctaagaatactctctacttgcagatgaacagcttaagggctgaggacacggccgtgtattactgtgcgaggtcgtattactatgatagtagtggttattactcacatgatgcttttgatatctggggccaagggacaatggtcaccgtctcaagc

SEQ ID NO: 263 - DNA, 324 bp, Artificial Sequence
  Synthetic Construct
gacatccagatgacccagtctccatcctccctgtctgcatctgtgggagacagagtcgccatcacttgccgcgcaagtcagagcatcgacacctatttaaattggtatcagcagaaaccagggaaagcccctaaactcctgatctatgctgcatccaagttggaagacggggtcccatcaagattcagtggcagtggaactgggacagatttcactctcaccatcagaagtctgcaacctgaagattttgcaagttatttctgtcaacagagctactctagtccagggatcactttcggccctgggaccaaggtggagatcaaa

SEQ ID NO: 264 - DNA, 366 bp, Artificial Sequence
  Synthetic Construct
gaagttcaattgttagagtctggtggcggtcttgttcagcctggtggttctttacgtctttcttgcgctgcttccggattcactttctctgattacgagatgcattgggttcgccaagctcctggtaaaggtttggagtgggtttcttctatctggccttctggtggccttactaagtatgctgaccccgttaaaggtcgcttcactatctctagagacaactctaagaatactctctacttgcagatgaacagcttaagggctgaggacacggccgtgtattactgtgcgagagattcctattactatgatagtagtggtgctcttggctactggggccagggaaccctggtcaccgtctcaagc

SEQ ID NO: 265 - DNA, 321 bp, Artificial Sequence
  Synthetic Construct
gacatccagatgacccagtctccttccaccctgtctgcatctgtaggagacagagtcaccatcacttgccgggccagtcagagtgttagtaactggttggcctggtatcagcagaaaccagggaaagcccctaagctcctgatctataaggcgtctagtttagaaagtggggtcccatcgaggttcagcggcagtggatctgggacagaattcactctcaccatcagcagcctgcagcctgatgattttgcaacttattactgcctacagtatgtgagttatcccctcacttttggcggagggaccaaggtggacatcaaa

SEQ ID NO: 266 - DNA, 372 bp, Artificial Sequence
  Synthetic Construct
gaagttcaattgttagagtctggtggcggtcttgttcagcctggtggttctttacgtctttcttgcgctgcttccggattcactttctcttattacgatatgtattgggttcgccaagctcctggtaaaggtttggagtgggtttctcgtatctattcttctggtggccatacttggtatgctgactccgttaaaggtcgcttcactatctctagagacaactctaagaatactctctacttgcagatgaacagcttaagggctgaggacacggctgtgtattactgtgcgaggcccgggtatagcagtggctggtacgatggcacctactttgactactggggccagggaaccctggtcaccgtctcaagc

SEQ ID NO: 267 - DNA, 321 bp, Artificial Sequence
  Synthetic Construct
gacatccagatgacccagtctccttccaccctgtctgcatctgttggcgacagagtcaccattacttgtcgggccagtcagagtattgatacttggctggcctggtatcggcagaaaccagggaaagcccctaatgtcgtaattcattccgcgtctactttacaaagtggcgtccccgcaaggttcagcggcagtggatttgggacagaatggactctcactatcaccaacctgcagcctgatgattttgccacctattattgccaacaatataagacttatccgttcacttttggccaggggacgaagctggagatcaag

SEQ ID NO: 268 - DNA, 357 bp, Artificial Sequence
  Synthetic Construct
gaagttcaattgttagagtctggtggcggtcttgttcagcctggtggttctttacgtctttcttgcgctgcttccggattcactttctctcattaccagatggagtgggttcgccaagctcctggtaaaggtttggagtgggtttcttctatctctccttctggtggctttacttcttatgctgactccgttaaaggtcgcttcactatctctagagacaactctaagaatactctctacttgcagatgaacagcttaagggctgaggacacagccgtgtattactgtacgagagagccggggaggttgtgggcttttgatatctggggccaagggacaatggtcaccgtctcaagc

SEQ ID NO: 269 - DNA, 321 bp, Artificial Sequence
  Synthetic Construct
gacatccagatgacccagtctccatctttcgtgtctgcatctgtcggagacagagtcaccatcacttgccgggcgagtcaggatattcgtaattggctagcctggtatcaacaggagtccgggaaagcccctcggctcctgatctctgctgcatccagtaggcacagtggcgtctcatctagattcagcggcagtggatctgggacagacttcaccctcaccatcaccagtctgcagcctgaagattcagcaacttatttttgtcaacaggctgacagttcccctcggacgttcggccaagggaccaaggtggaaatcaaa

SEQ ID NO: 270 - DNA, 345 bp, Artificial Sequence
  Synthetic Construct
caggtgcaactggtgcagtctggggctgaggtgaagaagcctggggcctcagtgaaggtctcctgcaaggcttctggatacaccttcaccggctactatatgcactgggtgcgacaggcccctggacaagggcttgagtggatgggatggatcaaccctaacagtggtggcacaaactatgcacagaagtttcagggcagggtcaccatgaccagggacacgtccatcaacacagcctacatggaactgagcaggctgagatctgacgacacggccgtgtattactgtgcggtctttggttcggggagttcttggggccagggaaccctggtcaccgtctcctca

SEQ ID NO: 271 - DNA, 321 bp, Artificial Sequence
  Synthetic Construct
gacatccagatgacccagtctccatcctcactgtctgcatctgtgggagacagagtcaccatcacttgtcgggcgagtcagggtattagcaattctttagcctggtttcagcagaaaccagggaaagcccctaagtccctgatctatgctgcatccagtttgcaaagtggggtcccatcaaagttcagcggcagtggatctgggacagatttcactctcaccatcagcagcctgcagcctgaagattttgcaacttattactgccaacaatataagagttacccgtacacatttggccaggggaccaagctggagatcaaa

SEQ ID NO: 272 - DNA, 345 bp, Artificial Sequence
  Synthetic Construct
caggtgcagctggtgcagtctggggctgaggtgaagaagcctggggcctcagtgaaggtctcctgcaaggcttctggaaacaccttcaccggctactatatacactgggttcgacaggcccctggacaagggcttgagtggatgggatggattaaacctagtactggtgacacaaactatgcacagaattttctggacagggtcaccatgaccagggacacgtccatcagcacagcctacatggaactcagcaggctgagatctgacgacacggccgtgtattactgtgcggtctttggttcggggagttcttggggccagggaaccctggtcaccgtctcctca

SEQ ID NO: 273 - DNA, 321 bp, Artificial Sequence
  Synthetic Construct
gacatccacatgacccagtctccatcctcactgtctgcatttgtaggagacagagtcaccatcacttgtcgggcgagtcagggcattagcaattatttagcctggtttcagcagaaaccagggaaagcccctaagtccctgatctatgctgcatccagtttgcaaagtggggtcccatcaaagttcagcggcagtggatctgggacagatttcactctcaccatcaacaacctgcagcctgaagattttgcaacttattactgccaacagtataagacttacccgtacacatttggccaggggaccaagctggagatcaaa

SEQ ID NO: 274 - DNA, 372 bp, Artificial Sequence
  Synthetic Construct
caggtgcagctggtggagtctgggggaggcgtggtccagcctgggaggtccctgagactctcctgtgcagcgtctggattcaccttcagtagctatggcatgcactgggtccgccaggctccaggcaaggggctggagtgggtggcagttatatggtatgatggaagtaataaatactatgcagactccgtgaagggccgattcaccatctccagagacaattccaagaacacgctgtatctgcaaatgaacagtctgagagccgaggacgcggctgtgtattactgtgcgagagaaggtggctggtacggcggggactactactacggtatggacgtctggggccaagggaccacggtcaccgtctcctca

SEQ ID NO: 275 - DNA, 321 bp, Artificial Sequence
  Synthetic Construct
gccatccagttgacccagtctccatcctccctgtctgcatctgtaggagacagagtcaccatcacttgccgggcaagtcagggcattagcagtgctttagcctggtatcagcagaaaccagggaaagctcctaagctcctgatctatgatgcctccagtttggaaagtggggtcccatcaaggttcagcggcagtggatctgggacagatttcactctcaccatcagcagcctgcagcctgaagattttgcaacttattactgtcatcagtttaataattacccattcactttcggccctgggaccaaagtggatatcaaa

SEQ ID NO: 276 - DNA, 366 bp, Artificial Sequence
  Synthetic Construct
gaagtgcagctgctggaatctggcggcggactggtgcagcctggcggatctctgagactgtcctgtgtggcctccggcttcaccttctccagctacgccatgtcctgggtgcgacaggctcctggcaagggcctggaatgggtgtccggcatctctggcaggggcggctctcctaactacgccgactctgtgaagggccggttcaccatctcccgggacaactccaagaacaccctgtacctccagatgaactccctgcgggccgaggacaccgccgtgtactactgtgctaaggacggcgacggctccggccctccctactactttgattactggggccagggcaccctcgtgaccgtgtcatct

SEQ ID NO: 277 - DNA, 321 bp, Artificial Sequence
  Synthetic Construct
gacatccagatgacccagtccccctccagcctgtctgcctctgtgggcgacagagtgaccatcacctgtcgggcctcccagggcatctcttcttggctggcctggtatcagcagaagcccgagaaggcccccaagtccctgatctacgccgccagctctctccagtctggcgtgccctccagattctccggctctggctctggcaccgactttaccctgaccatcagctccctccagcccgaggacttcgccacctactactgccagcagtacaactcctacccctacaccttcggccagggcaccaagctggaaatcaag

SEQ ID NO: 278 - DNA, 393 bp, Artificial Sequence
  Synthetic Construct
caggtgcagctgatggagtctgggggaggcgtggtccagcctgggaggtccctgagactctcctgtgcagcgtctggattcaccttcagtggctatggcatgcactgggtccgccaggctccagggaaggggctggagtgggtggcagttatatggtctgatggaagtaatagatactatacagactccgtgaagggccgattcaccatctccagagacaattccaagaacacgctgtctctgcaaatgaacagcctgagagccgaggacacggctgtgtattactgtgcgagagatagggggattactatggttcggggacttattataaaatactactactactacggtttggacgtctggggccaagggacctcggtcaccgtctcctca

SEQ ID NO: 279 - DNA, 318 bp, Artificial Sequence
  Synthetic Construct
gaaattgtgttgacacagtctccagccaccctgtctttgtctccaggggaaagagccaccctctcctgcagggccagtcagagtgttagcagctacttagcctggtaccaacagaaacctggccaggctcccaggctcctcatctatgatgcatccaacagggccactggcatcccagccaggttcagtggcagtgggtctgggacagacttcactctcaccatcagcagcctagagcctgaagattttgcagtttattactgtcagcagcgtagcaactggtggacgttcggccaagggaccaaggtggaaatcaaa

SEQ ID NO: 280 - DNA, 360 bp, Artificial Sequence
  Synthetic Construct
caggtgcagctggtggagtctgggggaggcgtggtccagcctgggaggtccctgagactctcctgtgcagcgtctggattcaccttcagtagctttggcatgcactgggtccgccaggctccaggcaaggggctggagtgggtggcagttatatactatgatggaagtaataaatactatgcagactccgtgaagggccgattcaccatctccagagacaattccaagaacacgctgtatctgcaaatgaacagcctgagagccgaggacacggctgtgtattactgtgcgagagatgacaactggaacgacggggactttgactactggggccagggaaccctggtcaccgtctcctca

SEQ ID NO: 281 - DNA, 321 bp, Artificial Sequence
  Synthetic Construct
gacatccagttgacccagtctccatccttcctgtctgcatctgtaggagacagagtcaccatcacttgccgggccagtcagggcattagtagttatttagcctggtatcagcaaaaaccagggaaagcccctaagctcctgatctatgctgcatccactttgcaaagtggggtcccatcaaggttcagcggcagtggatctgggacagaattcactctcacaatcagcagcctgcagcctgaagattttgcaacttattactgtcaacagcttaatagttaccctcggacgttcggccaagggaccaaggtggaaatcaaa

SEQ ID NO: 282 - DNA, 378 bp, Artificial Sequence
  Synthetic Construct
gaggtgcagctgttggagtctgggggaggcttggtacagcctggggagtccctgagactctcctgtgcagcctctggattcacctttaacagatttgtcatgagttgggtccgccaggctccagggaaggggctggagtgggtctcaactattagtggtagtggtggtagcacatactacgcagactccgtgaagggccggttcaccatctccagagacaattccaagaacacgctgtatctgcaaatgaacagcctgagagccgaggacacggccgtgtattactgtgcgaaagattttacgtattactatggttcggggaattattataactggttcgaccccaggggccagggaaccctggtcaccgtctcctca

SEQ ID NO: 283 - DNA, 321 bp, Artificial Sequence
  Synthetic Construct
gacatccagatgacccagtctccttccaccctgtctacatctgtaggagacagagtcaccatcacttgccgggccagtcagagtattagtagctggttggcctggtatcagcagaaaccagggaaagcccctaagctcctgatctataaggcgtctagtttagaaagtggggtcccatcaaggttcagcggcagtggatctgggacagaattcactctcaccatcagcagcctgcagcctgatgattttgcaacttattactgccaacagtataatagttattctcggacgttcggccaagggaccaaggtggaaatcaaa

SEQ ID NO: 284 - DNA, 363 bp, Artificial Sequence
  Synthetic Construct
caggtgcagctacagcagtggggcgcaggactgttgaagccttcggagaccctgtccctcacctgcgctgtctatggtgggtcctttagtggttactactggagctggatccgccagcccccagggaaggggctggagtggattggggaaatcaatcatagtggaggcaccaactacaacccgtccctcaagagtcgagtcaccatatcagtagacacgtccaagaaccacttctccctgaagctgagctctgtgaccgccgcggacacggctgtgtattactgtgcgagaactagtgactacgattactactactacggtatggacgtctggggccaagggaccacggtcaccgtctcctca

SEQ ID NO: 285 - DNA, 348 bp, Artificial Sequence
  Synthetic Construct
cagcctgtgctgactcagccaacttccctctcagcatctcctggagcatcagccagactcacctgcaccttgcgcagtggcatcaatcttggtcgctacaggatattctggtaccagcagaagccagagagccctccccggtatctcctgagctactactcagactcaagtaagcatcagggctctggagtccccagccgcttctctggatccaaagatgcttcgagcaatgcagggattttagtcatctctgggctccagtctgaggatgaggctgactattactgtatgatttggcacaggagtgctttgtttattttcggcagtggaaccaaggtcactgtccta

SEQ ID NO: 286 - DNA, 345 bp, Artificial Sequence
  Synthetic Construct
caggttcagctacagcagtctggacctgagctggtgaagcctggggcttcagtgaagttgtcctgcaaggcttctggttacaccttcacaagctacgagataaactggttgaagcagaggcctggacagggacttgagtggattggattgatttatcctagagatggagatactaagtacaatgagaagttcaagggcaaggccacattgactgcagacacatcctccagcacagcgtacatggagctccacagcctgacatctgaggactctgcggtctatttctgtgcaagacacaccccaggggctttctggggccaagggactctggtcactgtctctgca

SEQ ID NO: 287 - DNA, 336 bp, Artificial Sequence
  Synthetic Construct
gatgttgtgatgacccaaactcccctctccctgccggtcagtcttggagatcaagcctccatctcttgcagatctagtcagagccttgttcacagtaatggagacacctatttacattggtacctacagaagccaggccagtctccaaagctcctgatctacaaagtttccaaccgattttctggggtcccagacaggttcagtggcagtggatcagggacagatttcacactcaagatcagcagagtggaggctgaggatctggaaatttatttctgctctcaaagcacacatgttccgtacacgttcggaggggggaccaaactggaaataaaa

SEQ ID NO: 288 - DNA, 372 bp, Artificial Sequence
  Synthetic Construct
gacgtgaagctggtggagtctggggaaggcttagtgaagcccggagggtccctgaaactctcttgtgcagcctctggattcactttcagtaggtatgccatgtcttgggttcgccagactccagaaaagaggctggaatgggtcgcatatattagtagtggaggtgattacatccactatggagaaactgtgaagggccgattcaccatctccagagacaatgccaggaacaccctgtacctgcaaatgagcagtctgaagtctgaggacacagccatgtattactgtacaagagttctcttttattattacggcagtagctacgtcttttttgactactggggccaaggcaccactctcacagtctcctca

SEQ ID NO: 289 - DNA, 321 bp, Artificial Sequence
  Synthetic Construct
gatatccagatgacacagactacatcctccctgtcagtctctctgggagacagagtcaccatcagttgcagggcaagtcaggacatcagcaattttctaaactggtatcagcagaaaccagatggaactgttaatctcctgatctactacacatcaaaattacactcaggagtcccatcaaggttcagtggcggtgggtctggaagagattattctctcaccattaataacctggagcaagaagatattgcctcttacttttgccaacagggtcatacgcttccgtatacgttcggaggggggaccaagctggaaataaaa

SEQ ID NO: 290 - protein, 95 aa, Artificial Sequence
  Synthetic Construct
SIVVEWTNNTLPLEPCPKEQIIGLSRRIADENGKPRPAFSNALEPDFKALSIAVTGSGSCRHLQFIPVAPPSPGSSAAPATEVPDRDPEKSSEDD

SEQ ID NO: 291 - protein, 96 aa, Artificial Sequence
  Synthetic Construct
SIVVEWTNNTLPLEPCPKEQIAGLSRRIAEDDGKPRPAFSNALEPDFKATSITVTGSGSCRHLQFIPVVPPRRVPSEAPPTEVPDRDPEKSSEDDV

SEQ ID NO: 292 - protein, 183 aa, Artificial Sequence
  Synthetic Construct
ANAESGTYFDGTGFAKAVGGFKVGLDLLVEFEFRTWTGVLLGVSSQKMDGMGIEMIDEKLMFHVDNGAGRFTAIYDAGIPGHMCNGQWHKVTAKKIKNRLELVVDGNQVDAQSPNSASTSADTNDPVFVGGFPGQQFGLTTNIRFRGCIRSLKLTKGTGKPLEVNFAKALELRGVQPVSCPTT

SEQ ID NO: 293 - protein, 187 aa, Artificial Sequence
  Synthetic Construct
ANAQRGTYFDGTGFAKAVGGFKVGLDLLVEFEFRTTTTTGVLLGISSQKMDGMGIEMIDEKLMFHVDNGAGRFTAVYDAGVPGHLCDGQWHKVTANKIKHRIELTVDGNQVEAQSPNPASTSADTNDPVFVGGFPDDLKQFGLTTSIPFRGCIRSLKLTKGTGKPLEVNFAKALELRGVQPVSCPAN

SEQ ID NO: 294 - protein, 10 aa, Artificial Sequence
  Synthetic Construct
GGGGSGGGGS

SEQ ID NO: 295 - protein, 20 aa, Artificial Sequence
  Synthetic Construct
GFAKAVGGFKVGLDLLVEFE

SEQ ID NO: 296 - protein, 14 aa, Artificial Sequence
  Synthetic Construct
EPKSDKTHTSPPSP

SEQ ID NO: 297 - protein, 7 aa, Artificial Sequence
  Synthetic Construct
GQPKAAP

SEQ ID NO: 298 - protein, 5 aa, Artificial Sequence
  Synthetic Construct
TKGPS

SEQ ID NO: 299 - protein, 10 aa, Artificial Sequence
  Synthetic Construct
GGSGSSGSGG

SEQ ID NO: 300 - protein, 390 aa, Artificial Sequence
  Synthetic Construct
VQPQPVPTPAFPFPAPTMVHGPCVAESEPALLTGSKQFGLSRNSHIAIAFDDTKVKNRLTIELEVRTEAESGLLFYMARINHADFATVQLRNGFPYFSYDLGSGDTSTMIPTKINDGQWHKIKIVRVKQEGILYVDDASSQTISPKKADILDVVGILYVGGLPINYTTRRIGPVTYSLDGCVRNLHMEQAPVDLDQPTSSFHVGTCFANAESGTYFDGTGFAKAVGGFKVGLDLLVEFEFRTWTGVLLGVSSQKMDGMGIEMIDEKLMFHVDNGAGRFTAIYDAGIPGHMCNGQWHKVTAKKIKNRLELVVDGNQVDAQSPNSASTSADTNDPVFVGGFPGQQFGLTTNIRFRGCIRSLKLTKGTGKPLEVNFAKALELRGVQPVSCPTT

SEQ ID NO: 301 - protein, 391 aa, Artificial Sequence
  Synthetic Construct
QPEPVPTPAFPTPTPVLTHGPCAAESEPALLIGSKQFGLSRNSHIAIAFDDTKVKNRLTIELEVRTEAESGLLFYMARINHADFATVQLRNGLPYFSYDLGSGDTHTMIPTKINDGQWHKIKIMRSKQEGILYVDGNRTISPKKADILDVVGMLYVGGLPINYTTRRIGPVTYSIDGCVRNLHMAEAPADLEQPTSSFHVGTCFANAQRGTYFDGTGFAKAVGGFKVGLDLLVEFEFRTTTTTGVLLGISSQKMDGMGIEMIDEKLMFHVDNGAGRFTAVYDAGVPGHLCDGQWHKVTANKIKHRIELTVDGNQVEAQSPNPASTSADTNDPVFVGGFPDDLKQFGLTTSIPFRGCIRSLKLTKGTGKPLEVNFAKALELRGVQPVSCPAN

SEQ ID NO: 302 - protein, 11 aa, Artificial Sequence
  Synthetic Construct
DRDPEKSSEDD

SEQ ID NO: 303 - protein, 180 aa, Artificial Sequence
  Synthetic Construct
GDRAPARFKAKFVGDPALVLNDIHKKIALVKKLAFAFGDRNCSTITLQNITRGSIVVEWTNNTLPLEPCPKEQIAGLSRRIAEDDGKPRPAFSNALEPDFKATSITVTGSGSCRHLQFIPVVPPRRVPSEAPPTEVPDRDPEKSSEDDVYLHTVIPAVVVAAILLIAGIIAMICYRKKRK

SEQ ID NO: 304 - protein, 180 aa, Artificial Sequence
  Synthetic Construct
GDKAPARFKARLAGDPAPVVNDIHKKIALVKKLAFAFGDRNCSSITLQNITRGSIVVEWTNNTLPLEPCPKEQIIGLSRRIADENGKPRPAFSNALEPDFKALSIAVTGSGSCRHLQFIPVAPPSPGSSAAPATEVPDRDPEKSSEDDVYLHTVIPAVVVAAILLIAGIIAMICYRKKRK

SEQ ID NO: 305 - protein, 392 aa, Artificial Sequence
  Synthetic Construct
IQPEPVPTPAFPTPTPVLTHGPCAAESEPALLIGSKQFGLSRNSHIAIAFDDTKVKNRLTIELEVRTEAESGLLFYMARINHADFATVQLRNGLPYFSYDLGSGDTHTMIPTKINDGQWHKIKIMRSKQEGILYVDGNRTISPKKADILDVVGMLYVGGLPINYTTRRIGPVTYSIDGCVRNLHMAEAPADLEQPTSSFHVGTCFANAQRGTYFDGTGFAKAVGGFKVGLDLLVEFEFRTTTTTGVLLGISSQKMDGMGIEMIDEKLMFHVDNGAGRFTAVYDAGVPGHLCDGQWHKVTANKIKHRIELTVDGNQVEAQSPNPASTSADTNDPVFVGGFPDDLKQFGLTTSIPFRGCIRSLKLTKGTGKPLEVNFAKALELRGVQPVSCPAN

SEQ ID NO: 306 - DNA, 339 bp, Artificial Sequence
  Synthetic Construct
caagtacaactggttcaatcaggcgcagaagtcgtaaaacctggttccagcgtaaaagtcagttgtgaggctagtggattcaccttcaccgatagcgttattacatgggttcgtcagcgcccaggtcaagggctcgagtggattggggaaatttacccaggaagtggaaatttctactacaatgaaaaatttcaaggccgggtgaccatcactgctgataaaagcacttcaacagcctatatggaattgtccagcttgcgctccgaagacactgccgtttatttctgcgccatgcgtaggtcttcctggggacagggtacacttgtaactgtcagctct

SEQ ID NO: 307 - DNA, 75 bp, Artificial Sequence
  Synthetic Construct
caagtacaactggttcaatcaggcgcagaagtcgtaaaacctggttccagcgtaaaagtcagttgtgaggctagt

SEQ ID NO: 308 - DNA, 24 bp, Artificial Sequence
  Synthetic Construct
ggattcaccttcaccgatagcgtt

SEQ ID NO: 309 - DNA, 51 bp, Artificial Sequence
  Synthetic Construct
attacatgggttcgtcagcgcccaggtcaagggctcgagtggattggggaa

SEQ ID NO: 310 - DNA, 24 bp, Artificial Sequence
  Synthetic Construct
atttacccaggaagtggaaatttc

SEQ ID NO: 311 - DNA, 114 bp, Artificial Sequence
  Synthetic Construct
tactacaatgaaaaatttcaaggccgggtgaccatcactgctgataaaagcacttcaacagcctatatggaattgtccagcttgcgctccgaagacactgccgtttatttctgc

SEQ ID NO: 312 - DNA, 18 bp, Artificial Sequence
  Synthetic Construct
gccatgcgtaggtcttcc

SEQ ID NO: 313 - DNA, 33 bp, Artificial Sequence
  Synthetic Construct
tggggacagggtacacttgtaactgtcagctct

SEQ ID NO: 314 - protein, 113 aa, Artificial Sequence
  Synthetic Construct
QVQLVQSGAEVVKPGSSVKVSCEASGFTFTDSVITWVRQRPGQGLEWIGEIYPGSGNFYYNEKFQGRVTITADKSTSTAYMELSSLRSEDTAVYFCAMRRSSWGQGTLVTVSS

SEQ ID NO: 315 - protein, 25 aa, Artificial Sequence
  Synthetic Construct
QVQLVQSGAEVVKPGSSVKVSCEAS

SEQ ID NO: 316 - protein, 8 aa, Artificial Sequence
  Synthetic Construct
GFTFTDSV

SEQ ID NO: 317 - protein, 17 aa, Artificial Sequence
  Synthetic Construct
ITWVRQRPGQGLEWIGE

SEQ ID NO: 318 - protein, 8 aa, Artificial Sequence
  Synthetic Construct
IYPGSGNF

SEQ ID NO: 319 - protein, 38 aa, Artificial Sequence
  Synthetic Construct
YYNEKFQGRVTITADKSTSTAYMELSSLRSEDTAVYFC

SEQ ID NO: 320 - protein, 6 aa, Artificial Sequence
  Synthetic Construct
AMRRSS

SEQ ID NO: 321 - protein, 11 aa, Artificial Sequence
  Synthetic Construct
WGQGTLVTVSS

SEQ ID NO: 322 - DNA, 336 bp, Artificial Sequence
  Synthetic Construct
gacgtcgtaatgactcaaacacccctctctctttctgttacccccggacagcctgcttcaatcagttgtaaatcatcccaaaccatagttcattctaatagtaaaacttacctcgaatggtatctccaaaaacctggtcagtcaccacagctccttatttacaaggttagttccagattctctggcgtccctgaccgcttctctggctccggttcaggcaccgactttactctgaaaatctcacgggttgaagctgaagatgttggagtgtactactgcttccagggttctcacgtcccattgacctttggacagggaactaagctcgaaataaaa

SEQ ID NO: 323 - DNA, 78 bp, Artificial Sequence
  Synthetic Construct
gacgtcgtaatgactcaaacacccctctctctttctgttacccccggacagcctgcttcaatcagttgtaaatcatcc

SEQ ID NO: 324 - DNA, 33 bp, Artificial Sequence
  Synthetic Construct
caaaccatagttcattctaatagtaaaacttac

SEQ ID NO: 325 - DNA, 51 bp, Artificial Sequence
  Synthetic Construct
ctcgaatggtatctccaaaaacctggtcagtcaccacagctccttatttac

SEQ ID NO: 326 - DNA, 9 bp, Artificial Sequence
  Synthetic Construct
aaggttagt

SEQ ID NO: 327 - DNA, 108 bp, Artificial Sequence
  Synthetic Construct
tccagattctctggcgtccctgaccgcttctctggctccggttcaggcaccgactttactctgaaaatctcacgggttgaagctgaagatgttggagtgtactactgc

SEQ ID NO: 328 - DNA, 27 bp, Artificial Sequence
  Synthetic Construct
ttccagggttctcacgtcccattgacc

SEQ ID NO: 329 - DNA, 30 bp, Artificial Sequence
  Synthetic Construct
tttggacagggaactaagctcgaaataaaa

SEQ ID NO: 330 - protein, 112 aa, Artificial Sequence
  Synthetic Construct
DVVMTQTPLSLSVTPGQPASISCKSSQTIVHSNSKTYLEWYLQKPGQSPQLLIYKVSSRFSGVPDRFSGSGSGTDFTLKISRVEAEDVGVYYCFQGSHVPLTFGQGTKLEIK

SEQ ID NO: 331 - protein, 26 aa, Artificial Sequence
  Synthetic Construct
DVVMTQTPLSLSVTPGQPASISCKSS

SEQ ID NO: 332 - protein, 11 aa, Artificial Sequence
  Synthetic Construct
QTIVHSNSKTY

SEQ ID NO: 333 - protein, 17 aa, Artificial Sequence
  Synthetic Construct
LEWYLQKPGQSPQLLIY

SEQ ID NO: 334 - protein, 3 aa, Artificial Sequence
  Synthetic Construct
KVS

SEQ ID NO: 335 - protein, 36 aa, Artificial Sequence
  Synthetic Construct
SRFSGVPDRFSGSGSGTDFTLKISRVEAEDVGVYYC

SEQ ID NO: 336 - protein, 9 aa, Artificial Sequence
  Synthetic Construct
FQGSHVPLT

SEQ ID NO: 337 - protein, 10 aa, Artificial Sequence
  Synthetic Construct
FGQGTKLEIK

SEQ ID NO: 338 - DNA, 339 bp, Artificial Sequence; identical to SEQ ID NO: 306
  Synthetic Construct

SEQ ID NO: 339 - DNA, 75 bp, Artificial Sequence; identical to SEQ ID NO: 307
  Synthetic Construct

SEQ ID NO: 340 - DNA, 24 bp, Artificial Sequence
  Synthetic Construct
ggattcaccttcaccgatagcgtt

SEQ ID NO: 341 - DNA, 51 bp, Artificial Sequence; identical to SEQ ID NO: 309
  Synthetic Construct

SEQ ID NO: 342 - DNA, 24 bp, Artificial Sequence
  Synthetic Construct
atttacccaggaagtggaaatttc

SEQ ID NO: 343 - DNA, 114 bp, Artificial Sequence; identical to SEQ ID NO: 311
  Synthetic Construct

SEQ ID NO: 344 - DNA, 18 bp, Artificial Sequence
  Synthetic Construct
gccatgcgtaggtcttcc

SEQ ID NO: 345 - DNA, 33 bp, Artificial Sequence; identical to SEQ ID NO: 313
  Synthetic Construct

SEQ ID NO: 346 - protein, 113 aa, Artificial Sequence; identical to SEQ ID NO: 314
  Synthetic Construct

SEQ ID NO: 347 - protein, 25 aa, Artificial Sequence
  Synthetic Construct
QVQLVQSGAEVVKPGSSVKVSCEAS

SEQ ID NO: 348 - protein, 8 aa, Artificial Sequence
  Synthetic Construct
GFTFTDSV

SEQ ID NO: 349 - protein, 17 aa, Artificial Sequence
  Synthetic Construct
ITWVRQRPGQGLEWIGE

SEQ ID NO: 350 - protein, 8 aa, Artificial Sequence
  Synthetic Construct
IYPGSGNF

SEQ ID NO: 351 - protein, 38 aa, Artificial Sequence; identical to SEQ ID NO: 319
  Synthetic Construct

SEQ ID NO: 352 - protein, 6 aa, Artificial Sequence
  Synthetic Construct
AMRRSS

SEQ ID NO: 353 - protein, 11 aa, Artificial Sequence
  Synthetic Construct
WGQGTLVTVSS

SEQ ID NO: 354 - DNA, 336 bp, Artificial Sequence
  Synthetic Construct
gatgtggtgatgactcagacacccctgagtctcagcgtaacacctggtcaacccgcctctattagttgtcgaagctctcaaacaatcgtacatagtaatagtaaaacctatctcgaatggtatcttcagaaaccagggcagtctcctcaactccttatatacaaagtatccaacaggttttccggtgtacccgataggttttccggttccggctccggaactgactttaccctcaaaataagtcgagtggaggctgaggatgttggcgtttattattgctttcaggggtcacacgtacctcttaccttcggcgcaggcacaaaattggagattaaa

SEQ ID NO: 355 - DNA, 78 bp, Artificial Sequence
  Synthetic Construct
gatgtggtgatgactcagacacccctgagtctcagcgtaacacctggtcaacccgcctctattagttgtcgaagctct

SEQ ID NO: 356 - DNA, 33 bp, Artificial Sequence
  Synthetic Construct
caaacaatcgtacatagtaatagtaaaacctat

SEQ ID NO: 357 - DNA, 51 bp, Artificial Sequence
  Synthetic Construct
ctcgaatggtatcttcagaaaccagggcagtctcctcaactccttatatac

SEQ ID NO: 358 - DNA, 9 bp, Artificial Sequence
  Synthetic Construct
aaagtatcc

SEQ ID NO: 359 - DNA, 108 bp, Artificial Sequence
  Synthetic Construct
aacaggttttccggtgtacccgataggttttccggttccggctccggaactgactttaccctcaaaataagtcgagtggaggctgaggatgttggcgtttattattgc

SEQ ID NO: 360 - DNA, 27 bp, Artificial Sequence
  Synthetic Construct
tttcaggggtcacacgtacctcttacc

SEQ ID NO: 361 - DNA, 30 bp, Artificial Sequence
  Synthetic Construct
ttcggcgcaggcacaaaattggagattaaa

SEQ ID NO: 362 - protein, 112 aa, Artificial Sequence
  Synthetic Construct
DVVMTQTPLSLSVTPGQPASISCRSSQTIVHSNSKTYLEWYLQKPGQSPQLLIYKVSNRFSGVPDRFSGSGSGTDFTLKISRVEAEDVGVYYCFQGSHVPLTFGAGTKLEIK

SEQ ID NO: 363 - protein, 26 aa, Artificial Sequence
  Synthetic Construct
DVVMTQTPLSLSVTPGQPASISCRSS

SEQ ID NO: 364 - protein, 11 aa, Artificial Sequence
  Synthetic Construct
QTIVHSNSKTY

SEQ ID NO: 365 - protein, 17 aa, Artificial Sequence
  Synthetic Construct
LEWYLQKPGQSPQLLIY

SEQ ID NO: 366 - protein, 3 aa, Artificial Sequence
  Synthetic Construct
KVS

SEQ ID NO: 367 - protein, 36 aa, Artificial Sequence
  Synthetic Construct
NRFSGVPDRFSGSGSGTDFTLKISRVEAEDVGVYYC

SEQ ID NO: 368 - protein, 9 aa, Artificial Sequence
  Synthetic Construct
FQGSHVPLT

SEQ ID NO: 369 - protein, 10 aa, Artificial Sequence
  Synthetic Construct
FGAGTKLEIK

SEQ ID NO: 370 - DNA, 354 bp, Artificial Sequence
  Synthetic Construct
gaagttcaactggtcgagtctggaggaggcctcgtgaagccgggcggtagtttgcgcctctcttgtgccgcctcagggtttacgttctctagttatactatgagttgggtgcggcaggcaccgggaaaagggctggaatgggtggcctcaatctctagtagcggcagcaatacttattatcctgatagtgtgaaggggaggtttaccatctcacgggataacgctaagaacaacctgtatcttcaaatgaatagcctccgagcagaggatacagcactttactactgcgctcgctttgactatggcagcagtcttgatagttgggggcagggcaccttgcttacggtttcatcc

SEQ ID NO: 371 - DNA, 75 bp, Artificial Sequence
  Synthetic Construct
gaagttcaactggtcgagtctggaggaggcctcgtgaagccgggcggtagtttgcgcctctcttgtgccgcctca

SEQ ID NO: 372 - DNA, 24 bp, Artificial Sequence
  Synthetic Construct
gggtttacgttctctagttatact

SEQ ID NO: 373 - DNA, 51 bp, Artificial Sequence
  Synthetic Construct
atgagttgggtgcggcaggcaccgggaaaagggctggaatgggtggcctca

SEQ ID NO: 374 - DNA, 24 bp, Artificial Sequence
  Synthetic Construct
atctctagtagcggcagcaatact

SEQ ID NO: 375 - DNA, 114 bp, Artificial Sequence
  Synthetic Construct
tattatcctgatagtgtgaaggggaggtttaccatctcacgggataacgctaagaacaacctgtatcttcaaatgaatagcctccgagcagaggatacagcactttactactgc

SEQ ID NO: 376 - DNA, 33 bp, Artificial Sequence
  Synthetic Construct
gctcgctttgactatggcagcagtcttgatagt

SEQ ID NO: 377 - DNA, 33 bp, Artificial Sequence
  Synthetic Construct
tgggggcagggcaccttgcttacggtttcatcc

SEQ ID NO: 378 - protein, 118 aa, Artificial Sequence
  Synthetic Construct
EVQLVESGGGLVKPGGSLRLSCAASGFTFSSYTMSWVRQAPGKGLEWVASISSSGSNTYYPDSVKGRFTISRDNAKNNLYLQMNSLRAEDTALYYCARFDYGSSLDSWGQGTLLTVSS

SEQ ID NO: 379 - protein, 25 aa, Artificial Sequence
  Synthetic Construct
EVQLVESGGGLVKPGGSLRLSCAAS

SEQ ID NO: 380 - protein, 8 aa, Artificial Sequence
  Synthetic Construct
GFTFSSYT

SEQ ID NO: 381 - protein, 17 aa, Artificial Sequence
  Synthetic Construct
MSWVRQAPGKGLEWVAS

SEQ ID NO: 382 - protein, 8 aa, Artificial Sequence
  Synthetic Construct
ISSSGSNT

SEQ ID NO: 383 - protein, 38 aa, Artificial Sequence
  Synthetic Construct
YYPDSVKGRFTISRDNAKNNLYLQMNSLRAEDTALYYC

SEQ ID NO: 384 - protein, 11 aa, Artificial Sequence
  Synthetic Construct
ARFDYGSSLDS

SEQ ID NO: 385 - protein, 11 aa, Artificial Sequence
  Synthetic Construct
WGQGTLLTVSS

SEQ ID NO: 386 - DNA, 321 bp, Artificial Sequence
  Synthetic Construct
gagatcgttcttacccaatccccggatttcctttctgtgacccccaaagaaaaagtcacactcacctgccgagcaagccagtctattagtaacaatttgcactggtatcagcagaagagtgaccaatctcccaaactccttattaagtacgcctctcagtcaatatccggcatacctagccgcttttccggttctggtagtggcaccgactttactctcactatcaattcagtggaggctgaggatgccgccacgtatttttgtcagcaatcaaagagttggccccggacatttggagggggaactaagctggagattaag

SEQ ID NO: 387 - DNA, 78 bp, Artificial Sequence
  Synthetic Construct
gagatcgttcttacccaatccccggatttcctttctgtgacccccaaagaaaaagtcacactcacctgccgagcaagc

SEQ ID NO: 388 - DNA, 18 bp, Artificial Sequence
  Synthetic Construct
cagtctattagtaacaat

SEQ ID NO: 389 - DNA, 51 bp, Artificial Sequence
  Synthetic Construct
ttgcactggtatcagcagaagagtgaccaatctcccaaactccttattaag

SEQ ID NO: 390 - DNA, 9 bp, Artificial Sequence
  Synthetic Construct
tacgcctct

SEQ ID NO: 391 - DNA, 108 bp, Artificial Sequence
  Synthetic Construct
cagtcaatatccggcatacctagccgcttttccggttctggtagtggcaccgactttactctcactatcaattcagtggaggctgaggatgccgccacgtatttttgt

SEQ ID NO: 392 - DNA, 27 bp, Artificial Sequence
  Synthetic Construct
cagcaatcaaagagttggccccggaca

SEQ ID NO: 393 - DNA, 30 bp, Artificial Sequence
  Synthetic Construct
tttggagggggaactaagctggagattaag

SEQ ID NO: 394 - protein, 107 aa, Artificial Sequence
  Synthetic Construct
EIVLTQSPDFLSVTPKEKVTLTCRASQSISNNLHWYQQKSDQSPKLLIKYASQSISGIPSRFSGSGSGTDFTLTINSVEAEDAATYFCQQSKSWPRTFGGGTKLEIK

SEQ ID NO: 395 - protein, 26 aa, Artificial Sequence
  Synthetic Construct
EIVLTQSPDFLSVTPKEKVTLTCRAS

SEQ ID NO: 396 - protein, 6 aa, Artificial Sequence
  Synthetic Construct
QSISNN

SEQ ID NO: 397 - protein, 17 aa, Artificial Sequence
  Synthetic Construct
LHWYQQKSDQSPKLLIK

SEQ ID NO: 398 - protein, 3 aa, Artificial Sequence
  Synthetic Construct
YAS

SEQ ID NO: 399 - protein, 36 aa, Artificial Sequence
  Synthetic Construct
QSISGIPSRFSGSGSGTDFTLTINSVEAEDAATYFC

SEQ ID NO: 400 - protein, 9 aa, Artificial Sequence
  Synthetic Construct
QQSKSWPRT

SEQ ID NO: 401 - protein, 10 aa, Artificial Sequence
  Synthetic Construct
FGGGTKLEIK

SEQ ID NO: 402 - DNA, 354 bp, Artificial Sequence; identical to SEQ ID NO: 370
  Synthetic Construct

SEQ ID NO: 403 - DNA, 75 bp, Artificial Sequence; identical to SEQ ID NO: 371
  Synthetic Construct

SEQ ID NO: 404 - DNA, 24 bp, Artificial Sequence
  Synthetic Construct
gggtttacgttctctagttatact

SEQ ID NO: 405 - DNA, 51 bp, Artificial Sequence; identical to SEQ ID NO: 373
  Synthetic Construct

SEQ ID NO: 406 - DNA, 24 bp, Artificial Sequence
  Synthetic Construct
atctctagtagcggcagcaatact

SEQ ID NO: 407 - DNA, 114 bp, Artificial Sequence; identical to SEQ ID NO: 375
  Synthetic Construct

SEQ ID NO: 408 - DNA, 33 bp, Artificial Sequence; identical to SEQ ID NO: 376
  Synthetic Construct

SEQ ID NO: 409 - DNA, 33 bp, Artificial Sequence; identical to SEQ ID NO: 377
  Synthetic Construct

SEQ ID NO: 410 - protein, 118 aa, Artificial Sequence; identical to SEQ ID NO: 378
  Synthetic Construct

SEQ ID NO: 411 - protein, 25 aa, Artificial Sequence
  Synthetic Construct
EVQLVESGGGLVKPGGSLRLSCAAS

SEQ ID NO: 412 - protein, 8 aa, Artificial Sequence
  Synthetic Construct
GFTFSSYT

SEQ ID NO: 413 - protein, 17 aa, Artificial Sequence
  Synthetic Construct
MSWVRQAPGKGLEWVAS

SEQ ID NO: 414 - protein, 8 aa, Artificial Sequence
  Synthetic Construct
ISSSGSNT

SEQ ID NO: 415 - protein, 38 aa, Artificial Sequence; identical to SEQ ID NO: 383
  Synthetic Construct

SEQ ID NO: 416 - protein, 11 aa, Artificial Sequence
  Synthetic Construct
ARFDYGSSLDS

SEQ ID NO: 417 - protein, 11 aa, Artificial Sequence
  Synthetic Construct
WGQGTLLTVSS

SEQ ID NO: 418 - DNA, 321 bp, Artificial Sequence
  Synthetic Construct
gaaattgtgcttacccagtccccagacttcctgtccgtgacccctaaagagaaggtgacactgacttgcagggcctcacaatccattggcaataaccttcactggtatcagcagaagtccgaccagtctccgaaactcctcatcaagtatgccagccagtcaattagcggaataccgtctcggtttagcggatctgggtctggtactgacttcacgctgacgatcaatagcgtggaagcggaggacgccgccacctatttctgccagcaatctaagtcctggccgagaacgttcggaggcggtactaaacttgagatcaag

SEQ ID NO: 419 - DNA, 78 bp, Artificial Sequence
  Synthetic Construct
gaaattgtgcttacccagtccccagacttcctgtccgtgacccctaaagagaaggtgacactgacttgcagggcctca

SEQ ID NO: 420 - DNA, 18 bp, Artificial Sequence
  Synthetic Construct
caatccattggcaataac

SEQ ID NO: 421 - DNA, 51 bp, Artificial Sequence
  Synthetic Construct
cttcactggtatcagcagaagtccgaccagtctccgaaactcctcatcaag

SEQ ID NO: 422 - DNA, 9 bp, Artificial Sequence
  Synthetic Construct
tatgccagc

SEQ ID NO: 423 - DNA, 108 bp, Artificial Sequence
  Synthetic Construct
cagtcaattagcggaataccgtctcggtttagcggatctgggtctggtactgacttcacgctgacgatcaatagcgtggaagcggaggacgccgccacctatttctgc

SEQ ID NO: 424 - DNA, 27 bp, Artificial Sequence
  Synthetic Construct
cagcaatctaagtcctggccgagaacg

SEQ ID NO: 425 - DNA, 30 bp, Artificial Sequence
  Synthetic Construct
ttcggaggcggtactaaacttgagatcaag

SEQ ID NO: 426 - protein, 107 aa, Artificial Sequence
  Synthetic Construct
EIVLTQSPDFLSVTPKEKVTLTCRASQSIGNNLHWYQQKSDQSPKLLIKYASQSISGIPSRFSGSGSGTDFTLTINSVEAEDAATYFCQQSKSWPRTFGGGTKLEIK

SEQ ID NO: 427 - protein, 26 aa, Artificial Sequence
  Synthetic Construct
EIVLTQSPDFLSVTPKEKVTLTCRAS

SEQ ID NO: 428 - protein, 6 aa, Artificial Sequence
  Synthetic Construct
QSIGNN

SEQ ID NO: 429 - protein, 17 aa, Artificial Sequence
  Synthetic Construct
LHWYQQKSDQSPKLLIK

SEQ ID NO: 430 - protein, 3 aa, Artificial Sequence
  Synthetic Construct
YAS

SEQ ID NO: 431 - protein, 36 aa, Artificial Sequence; identical to SEQ ID NO: 399
  Synthetic Construct

SEQ ID NO: 432 - protein, 9 aa, Artificial Sequence
  Synthetic Construct
QQSKSWPRT

SEQ ID NO: 433 - protein, 10 aa, Artificial Sequence
  Synthetic Construct
FGGGTKLEIK

SEQ ID NO: 434 - DNA, 354 bp, Artificial Sequence
  Synthetic Construct
gaggtacagctcgtcgaaagtggcggcggtcttgtcaagccgggaggaagtttgcgcctgtcctgtgcagcatccggattcacgttttcttcttatacgatgagttgggtccggcaggcaccggggaaaggattggaatgggttgcgtctattagtagctctggatctaacacatactacccagactcagttaaaggtcgcttcacgataagtcgggacaacgctaaaaataacctgtatttgcaaatgaacagcttgcgagctgaggacaccgccctctactactgtgcccgatttgattatggatcaagtttggattcatggggccaagggaccctgctcacagtaagctct

SEQ ID NO: 435 - DNA, 75 bp, Artificial Sequence
  Synthetic Construct
gaggtacagctcgtcgaaagtggcggcggtcttgtcaagccgggaggaagtttgcgcctgtcctgtgcagcatcc

SEQ ID NO: 436 - DNA, 24 bp, Artificial Sequence
  Synthetic Construct
ggattcacgttttcttcttatacg

SEQ ID NO: 437 - DNA, 51 bp, Artificial Sequence
  Synthetic Construct
atgagttgggtccggcaggcaccggggaaaggattggaatgggttgcgtct

SEQ ID NO: 438 - DNA, 24 bp, Artificial Sequence
  Synthetic Construct
attagtagctctggatctaacaca

SEQ ID NO: 439 - DNA, 114 bp, Artificial Sequence
  Synthetic Construct
tactacccagactcagttaaaggtcgcttcacgataagtcgggacaacgctaaaaataacctgtatttgcaaatgaacagcttgcgagctgaggacaccgccctctactactgt

SEQ ID NO: 440 - DNA, 33 bp, Artificial Sequence
  Synthetic Construct
gcccgatttgattatggatcaagtttggattca

SEQ ID NO: 441 - DNA, 33 bp, Artificial Sequence
  Synthetic Construct
tggggccaagggaccctgctcacagtaagctct

SEQ ID NO: 442 - protein, 118 aa, Artificial Sequence; identical to SEQ ID NO: 378
  Synthetic Construct

SEQ ID NO: 443 - protein, 25 aa, Artificial Sequence
  Synthetic Construct
EVQLVESGGGLVKPGGSLRLSCAAS

SEQ ID NO: 444 - protein, 8 aa, Artificial Sequence
  Synthetic Construct
GFTFSSYT

SEQ ID NO: 445 - protein, 17 aa, Artificial Sequence
  Synthetic Construct
MSWVRQAPGKGLEWVAS

SEQ ID NO: 446 - protein, 8 aa, Artificial Sequence
  Synthetic Construct
ISSSGSNT

SEQ ID NO: 447 - protein, 38 aa, Artificial Sequence; identical to SEQ ID NO: 383
  Synthetic Construct

SEQ ID NO: 448 - protein, 11 aa, Artificial Sequence
  Synthetic Construct
ARFDYGSSLDS

SEQ ID NO: 449 - protein, 11 aa, Artificial Sequence
  Synthetic Construct
WGQGTLLTVSS

SEQ ID NO: 450 - DNA, 321 bp, Artificial Sequence
  Synthetic Construct
gaaatcgttcttactcagtccccggattttttgagtgtaacgcctaaagagaaggtgaccctgtcctgccgcgcttcccaatctatatcaaactatcttcattggtaccagcaaaaaagcgaccagtccccgaaactgctcatcaaatacgctagccaatcaataagcggcatccctagcaggttttccggtagcggtagtggcacagacttcacattgagcataaacagcgtggaagccgaggatgcagcaacatacttttgccaacagagcaagtcctggccgaggacgttcggtgggggcaccaaattggaaataaag

SEQ ID NO: 451 - DNA, 78 bp, Artificial Sequence
  Synthetic Construct
gaaatcgttcttactcagtccccggattttttgagtgtaacgcctaaagagaaggtgaccctgtcctgccgcgcttcc

SEQ ID NO: 452 - DNA, 18 bp, Artificial Sequence
  Synthetic Construct
caatctatatcaaactat

SEQ ID NO: 453 - DNA, 51 bp, Artificial Sequence
  Synthetic Construct
cttcattggtaccagcaaaaaagcgaccagtccccgaaactgctcatcaaa

SEQ ID NO: 454 - DNA, 9 bp, Artificial Sequence
  Synthetic Construct
tacgctagc

SEQ ID NO: 455 - DNA, 108 bp, Artificial Sequence
  Synthetic Construct
caatcaataagcggcatccctagcaggttttccggtagcggtagtggcacagacttcacattgagcataaacagcgtggaagccgaggatgcagcaacatacttttgc

SEQ ID NO: 456 - DNA, 27 bp, Artificial Sequence
  Synthetic Construct
caacagagcaagtcctggccgaggacg

SEQ ID NO: 457 - DNA, 30 bp, Artificial Sequence
  Synthetic Construct
ttcggtgggggcaccaaattggaaataaag

SEQ ID NO: 458 - protein, 107 aa, Artificial Sequence
  Synthetic Construct
EIVLTQSPDFLSVTPKEKVTLSCRASQSISNYLHWYQQKSDQSPKLLIKYASQSISGIPSRFSGSGSGTDFTLSINSVEAEDAATYFCQQSKSWPRTFGGGTKLEIK

SEQ ID NO: 459 - protein, 26 aa, Artificial Sequence
  Synthetic Construct
EIVLTQSPDFLSVTPKEKVTLSCRAS

SEQ ID NO: 460 - protein, 6 aa, Artificial Sequence
  Synthetic Construct
QSISNY

SEQ ID NO: 461 - protein, 17 aa, Artificial Sequence
  Synthetic Construct
LHWYQQKSDQSPKLLIK

SEQ ID NO: 462 - protein, 3 aa, Artificial Sequence
  Synthetic Construct
YAS

SEQ ID NO: 463 - protein, 36 aa, Artificial Sequence
  Synthetic Construct
QSISGIPSRFSGSGSGTDFTLSINSVEAEDAATYFC

SEQ ID NO: 464 - protein, 9 aa, Artificial Sequence
  Synthetic Construct
QQSKSWPRT

SEQ ID NO: 465 - protein, 10 aa, Artificial Sequence
  Synthetic Construct
FGGGTKLEIK

SEQ ID NO: 466 - DNA, 354 bp, Artificial Sequence
  Synthetic Construct
gaggtccaacttgttgaatccggtggagggctggtgcagcctggtggatccctccgcctttcctgtgcagcatcaggttttactttttcctcatacaccatgtcttgggttcgccaggctccagggaaaggattggaatgggtggcaactatcagtagtagcggggacaatacatactatcccgattccgtgaaagggagatttacgatttcacgcgacaacagcaaaaataccctttacctgcaaatgagttccttgcgggccgaggacactgccctctactactgcgctcgcttcgattacggttccagcctggactcatggggtcaagggactacactgactgtttcttcc

SEQ ID NO: 467 - DNA, 75 bp, Artificial Sequence
  Synthetic Construct
gaggtccaacttgttgaatccggtggagggctggtgcagcctggtggatccctccgcctttcctgtgcagcatca

SEQ ID NO: 468 - DNA, 24 bp, Artificial Sequence
  Synthetic Construct
ggttttactttttcctcatacacc

SEQ ID NO: 469 - DNA, 51 bp, Artificial Sequence
  Synthetic Construct
atgtcttgggttcgccaggctccagggaaaggattggaatgggtggcaact

SEQ ID NO: 470 - DNA, 24 bp, Artificial Sequence
  Synthetic Construct
atcagtagtagcggggacaataca

SEQ ID NO: 471 - DNA, 114 bp, Artificial Sequence
  Synthetic Construct
tactatcccgattccgtgaaagggagatttacgatttcacgcgacaacagcaaaaataccctttacctgcaaatgagttccttgcgggccgaggacactgccctctactactgc

SEQ ID NO: 472 - DNA, 33 bp, Artificial Sequence
  Synthetic Construct
gctcgcttcgattacggttccagcctggactca

SEQ ID NO: 473 - DNA, 33 bp, Artificial Sequence
  Synthetic Construct
tggggtcaagggactacactgactgtttcttcc

SEQ ID NO: 474 - protein, 118 aa, Artificial Sequence
  Synthetic Construct
EVQLVESGGGLVQPGGSLRLSCAASGFTFSSYTMSWVRQAPGKGLEWVATISSSGDNTYYPDSVKGRFTISRDNSKNTLYLQMSSLRAEDTALYYCARFDYGSSLDSWGQGTTLTVSS

SEQ ID NO: 475 - protein, 25 aa, Artificial Sequence [sequence omitted]

SEQ ID NO: 476 - protein, 8 aa, Artificial Sequence
  Synthetic Construct
GFTFSSYT

SEQ ID NO: 477 - protein, 17 aa, Artificial Sequence
  Synthetic Construct
MSWVRQAPGKGLEWVAT

SEQ ID NO: 478 - protein, 8 aa, Artificial Sequence
  Synthetic Construct
ISSSGDNT

SEQ ID NO: 479 - protein, 38 aa, Artificial Sequence
  Synthetic Construct
YYPDSVKGRFTISRDNSKNTLYLQMSSLRAEDTALYYC

SEQ ID NO: 480 - protein, 11 aa, Artificial Sequence
  Synthetic Construct
ARFDYGSSLDS

SEQ ID NO: 481 - protein, 11 aa, Artificial Sequence
  Synthetic Construct
WGQGTTLTVSS

SEQ ID NO: 482 - DNA, 321 bp, Artificial Sequence
  Synthetic Construct
gagatcgtgctcacccaatctcctgacttccttagcgttacaccaggggagaaagtaactcttacgtgccgggcctcccagagcatctccaattatttgcattggtaccagcaaaagagtgaccagagccctaagctgctcatcaaatacgcatcacagagtattagcggcgttccctcacggttctctggctccggttccggtacagacttcactttgacgatttcaagtgtagaggccgaggacttcgcaacttacttttgtcagcaaagcaaatcctggcctcgaactttcggcgggggtacaaaactcgaaatcaag

SEQ ID NO: 483 - DNA, 78 bp, Artificial Sequence
  Synthetic Construct
gagatcgtgctcacccaatctcctgacttccttagcgttacaccaggggagaaagtaactcttacgtgccgggcctcc

SEQ ID NO: 484 - DNA, 18 bp, Artificial Sequence
  Synthetic Construct
cagagcatctccaattat

SEQ ID NO: 485 - DNA, 51 bp, Artificial Sequence
  Synthetic Construct
ttgcattggtaccagcaaaagagtgaccagagccctaagctgctcatcaaa

SEQ ID NO: 486 - DNA, 9 bp, Artificial Sequence
  Synthetic Construct
tacgcatca

SEQ ID NO: 487 - DNA, 108 bp, Artificial Sequence
  Synthetic Construct
cagagtattagcggcgttccctcacggttctctggctccggttccggtacagacttcactttgacgatttcaagtgtagaggccgaggacttcgcaacttacttttgt

SEQ ID NO: 488 - DNA, 27 bp, Artificial Sequence
  Synthetic Construct
cagcaaagcaaatcctggcctcgaact

SEQ ID NO: 489 - DNA, 30 bp, Artificial Sequence
  Synthetic Construct
ttcggcgggggtacaaaactcgaaatcaag

SEQ ID NO: 490 - protein, 107 aa, Artificial Sequence
  Synthetic Construct
EIVLTQSPDFLSVTPGEKVTLTCRASQSISNYLHWYQQKSDQSPKLLIKYASQSISGVPSRFSGSGSGTDFTLTISSVEAEDFATYFCQQSKSWPRTFGGGTKLEIK

SEQ ID NO: 491 - protein, 26 aa, Artificial Sequence
  Synthetic Construct
EIVLTQSPDFLSVTPGEKVTLTCRAS

SEQ ID NO: 492 - protein, 6 aa, Artificial Sequence
  Synthetic Construct
QSISNY

SEQ ID NO: 493 - protein, 17 aa, Artificial Sequence
  Synthetic Construct
LHWYQQKSDQSPKLLIK

SEQ ID NO: 494 - protein, 3 aa, Artificial Sequence
  Synthetic Construct
YAS

SEQ ID NO: 495 - protein, 36 aa, Artificial Sequence
  Synthetic Construct
QSISGVPSRFSGSGSGTDFTLTISSVEAEDFATYFC

SEQ ID NO: 496 - protein, 9 aa, Artificial Sequence
  Synthetic Construct
QQSKSWPRT

SEQ ID NO: 497 - protein, 10 aa, Artificial Sequence
  Synthetic Construct
FGGGTKLEIK

SEQ ID NO: 498 - protein, 571 aa, Artificial Sequence
  Synthetic Construct
EVQLVESGGGLVKPGGSLRLSCAASGFTFSSYTMSWVRQAPGKGLEWVASISSSGSNTYYPDSVKGRFTISRDNAKNNLYLQMNSLRAEDTALYYCARFDYGSSLDSWGQGTLLTVSSDKTHTEVQLVESGGGLVKPGGSLRLSCAASGFTFSSYTMSWVRQAPGKGLEWVASISSSGSNTYYPDSVKGRFTISRDNAKNNLYLQMNSLRAEDTALYYCARFDYGSSLDSWGQGTLLTVSSDKTHTASTKGPSVFPLAPSSKSTSGGTAALGCLVKDYFPEPVTVSWNSGALTSGVHTFPAVLQSSGSLSSVVTVPSSSLGTQTYICNVNHKPSNTKVDKKVEPKSCDKTHTCPPCPAPELLGGPSVFLFPPKPKDTLYITREPEVTCVVVDVSHEDPEVKFNWYVDGVEVHNAKTKPREEQYNNASRVVSVLTVLHQDWLNGKEYKCKVSNKALPAPIEKTISKAKGQPREPQVYTLPPCRDELTKNQVSLWCLVKGFYPSDIAVEWESNGQPENNYKTTPPVLDSDGSFFKKLTVDKSRWQQGNVFSCSVMHEALHNHYTQKSLSLSPG

SEQ ID NO: 499 - protein, 440 aa, Artificial Sequence
  Synthetic Construct
QVQLVQSGAEVVKPGSSVKVSCEASGFTFTDSVITWVRQRPGQGLEWIGEIYPGSGNFYYNEKFQGRVTITADKSTSTAYMELSSLRSEDTAVYFCAMRRSSWGQGTLVTVSSASTKGPSVFPLAPSSKSTSGGTAALGCLVKDYFPEPVTVSWNSGALTSGVHTFPAVLQSSGSLSSVVTVPSSSLGTQTYICNVNHKPSNTKVDKKVEPKSCDKTHTCPPCPAPELLGGPSVFLFPPKPKDTLYITREPEVTCVVVDVSHEDPEVKFNWYVDGVEVHNAKTKPREEQYNNASRVVSVLTVLHQDWLNGKEYKCKVSNKALPAPIEKTISKAKGQPREPQVCTLPPSRDELTKNQVSLSCAVKGFYPSDIAVEWESNGQPENNYKTTPPVLDSDGSFFLVSKLTVDKSRWQQGNVFSCSVMHEALHNRFTQKSLSLSPG

SEQ ID NO: 500 - protein, 331 aa, Artificial Sequence
  Synthetic Construct
EIVLTQSPDFLSVTPKEKVTLTCRASQSISNNLHWYQQKSDQSPKLLIKYASQSISGIPSRFSGSGSGTDFTLTINSVEAEDAATYFCQQSKSWPRTFGGGTKLEIKDKTHTEIVLTQSPDFLSVTPKEKVTLTCRASQSISNNLHWYQQKSDQSPKLLIKYASQSISGIPSRFSGSGSGTDFTLTINSVEAEDAATYFCQQSKSWPRTFGGGTKLEIKDKTHTRTVAAPSVFIFPPSDEQLKSGTASVVCLLNNFYPREAKVQWKVDNALQSGNSQESVTEQDSKDSTYSLSSTLTLSKADYEKHKVYACEVTHQGLSSPVTKSFNRGEC

SEQ ID NO: 501 - protein, 219 aa, Artificial Sequence
  Synthetic Construct
DVVMTQTPLSLSVTPGQPASISCKSSQTIVHSNSKTYLEWYLQKPGQSPQLLIYKVSSRFSGVPDRFSGSGSGTDFTLKISRVEAEDVGVYYCFQGSHVPLTFGQGTKLEIKRTVAAPSVFIFPPSDEQLKSGTASVVCLLNNFYPREAKVQWKVDNALQSGNSQESVTEQDSKDSTYSLSSTLTLSKADYEKHKVYACEVTHQGLSSPVTKSFNRGEC

SEQ ID NO: 502 - protein, 571 aa, Artificial Sequence; identical to SEQ ID NO: 498
  Synthetic Construct

SEQ ID NO: 503 - protein, 440 aa, Artificial Sequence; identical to SEQ ID NO: 499
  Synthetic Construct

SEQ ID NO: 504 - protein, 331 aa, Artificial Sequence
  Synthetic Construct
EIVLTQSPDFLSVTPKEKVTLSCRASQSISNYLHWYQQKSDQSPKLLIKYASQSISGIPSRFSGSGSGTDFTLSINSVEAEDAATYFCQQSKSWPRTFGGGTKLEIKDKTHTEIVLTQSPDFLSVTPKEKVTLTCRASQSISNNLHWYQQKSDQSPKLLIKYASQSISGIPSRFSGSGSGTDFTLTINSVEAEDAATYFCQQSKSWPRTFGGGTKLEIKDKTHTRTVAAPSVFIFPPSDEQLKSGTASVVCLLNNFYPREAKVQWKVDNALQSGNSQESVTEQDSKDSTYSLSSTLTLSKADYEKHKVYACEVTHQGLSSPVTKSFNRGEC

SEQ ID NO: 505 - protein, 219 aa, Artificial Sequence; identical to SEQ ID NO: 501
  Synthetic Construct

SEQ ID NO: 506 - protein, 571 aa, Artificial Sequence
  Synthetic Construct
EVQLVESGGGLVKPGGSLRLSCAASGFTFSSYTMSWVRQAPGKGLEWVASISSSGSNTYYPDSVKGRFTISRDNAKNNLYLQMNSLRAEDTALYYCARFDYGSSLDSWGQGTLLTVSSDKTHTEVQLVESGGGLVQPGGSLRLSCAASGFTFSSYTMSWVRQAPGKGLEWVATISSSGDNTYYPDSVKGRFTISRDNSKNTLYLQMSSLRAEDTALYYCARFDYGSSLDSWGQGTTLTVSSDKTHTASTKGPSVFPLAPSSKSTSGGTAALGCLVKDYFPEPVTVSWNSGALTSGVHTFPAVLQSSGSLSSVVTVPSSSLGTQTYICNVNHKPSNTKVDKKVEPKSCDKTHTCPPCPAPELLGGPSVFLFPPKPKDTLYITREPEVTCVVVDVSHEDPEVKFNWYVDGVEVHNAKTKPREEQYNNASRVVSVLTVLHQDWLNGKEYKCKVSNKALPAPIEKTISKAKGQPREPQVYTLPPCRDELTKNQVSLWCLVKGFYPSDIAVEWESNGQPENNYKTTPPVLDSDGSFFKKLTVDKSRWQQGNVFSCSVMHEALHNHYTQKSLSLSPG

SEQ ID NO: 507 - protein, 440 aa, Artificial Sequence; identical to SEQ ID NO: 499
  Synthetic Construct

SEQ ID NO: 508 - protein, 331 aa, Artificial Sequence
  Synthetic Construct
EIVLTQSPDFLSVTPGEKVTLTCRASQSISNYLHWYQQKSDQSPKLLIKYASQSISGVPSRFSGSGSGTDFTLTISSVEAEDFATYFCQQSKSWPRTFGGGTKLEIKDKTHTEIVLTQSPDFLSVTPKEKVTLTCRASQSIGNNLHWYQQKSDQSPKLLIKYASQSISGIPSRFSGSGSGTDFTLTINSVEAEDAATYFCQQSKSWPRTFGGGTKLEIKDKTHTRTVAAPSVFIFPPSDEQLKSGTASVVCLLNNFYPREAKVQWKVDNALQSGNSQESVTEQDSKDSTYSLSSTLTLSKADYEKHKVYACEVTHQGLSSPVTKSFNRGEC

SEQ ID NO: 509 - protein, 219 aa, Artificial Sequence; identical to SEQ ID NO: 501
  Synthetic Construct

SEQ ID NO: 510 - protein, 571 aa, Artificial Sequence; identical to SEQ ID NO: 498
  Synthetic Construct

SEQ ID NO: 511 - protein, 440 aa, Artificial Sequence; identical to SEQ ID NO: 499
  Synthetic Construct

SEQ ID NO: 512 - protein, 331 aa, Artificial Sequence
  Synthetic Construct
EIVLTQSPDFLSVTPKEKVTLTCRASQSIGNNLHWYQQKSDQSPKLLIKYASQSISGIPSRFSGSGSGTDFTLTINSVEAEDAATYFCQQSKSWPRTFGGGTKLEIKDKTHTEIVLTQSPDFLSVTPKEKVTLSCRASQSISNYLHWYQQKSDQSPKLLIKYASQSISGIPSRFSGSGSGTDFTLSINSVEAEDAATYFCQQSKSWPRTFGGGTKLEIKDKTHTRTVAAPSVFIFPPSDEQLKSGTASVVCLLNNFYPREAKVQWKVDNALQSGNSQESVTEQDSKDSTYSLSSTLTLSKADYEKHKVYACEVTHQGLSSPVTKSFNRGEC

SEQ ID NO: 513 - protein, 219 aa, Artificial Sequence; identical to SEQ ID NO: 501
  Synthetic Construct

SEQ ID NO: 514 - protein, 571 aa, Artificial Sequence
  Synthetic Construct
EVQLVESGGGLVQPGGSLRLSCAASGFTFSSYTMSWVRQAPGKGLEWVATISSSGDNTYYPDSVKGRFTISRDNSKNTLYLQMSSLRAEDTALYYCARFDYGSSLDSWGQGTTLTVSSDKTHTEVQLVESGGGLVKPGGSLRLSCAASGFTFSSYTMSWVRQAPGKGLEWVASISSSGSNTYYPDSVKGRFTISRDNAKNNLYLQMNSLRAEDTALYYCARFDYGSSLDSWGQGTLLTVSSDKTHTASTKGPSVFPLAPSSKSTSGGTAALGCLVKDYFPEPVTVSWNSGALTSGVHTFPAVLQSSGSLSSVVTVPSSSLGTQTYICNVNHKPSNTKVDKKVEPKSCDKTHTCPPCPAPELLGGPSVFLFPPKPKDTLYITREPEVTCVVVDVSHEDPEVKFNWYVDGVEVHNAKTKPREEQYNNASRVVSVLTVLHQDWLNGKEYKCKVSNKALPAPIEKTISKAKGQPREPQVYTLPPCRDELTKNQVSLWCLVKGFYPSDIAVEWESNGQPENNYKTTPPVLDSDGSFFKKLTVDKSRWQQGNVFSCSVMHEALHNHYTQKSLSLSPG

SEQ ID NO: 515 - protein, 440 aa, Artificial Sequence; identical to SEQ ID NO: 499
  Synthetic Construct

SEQ ID NO: 516 - protein, 331 aa, Artificial Sequence
  Synthetic Construct
EIVLTQSPDFLSVTPKEKVTLTCRASQSISNNLHWYQQKSDQSPKLLIKYASQSISGIPSRFSGSGSGTDFTLTINSVEAEDAATYFCQQSKSWPRTFGGGTKLEIKDKTHTEIVLTQSPDFLSVTPGEKVTLTCRASQSISNYLHWYQQKSDQSPKLLIKYASQSISGVPSRFSGSGSGTDFTLTISSVEAEDFATYFCQQSKSWPRTFGGGTKLEIKDKTHTRTVAAPSVFIFPPSDEQLKSGTASVVCLLNNFYPREAKVQWKVDNALQSGNSQESVTEQDSKDSTYSLSSTLTLSKADYEKHKVYACEVTHQGLSSPVTKSFNRGEC

SEQ ID NO: 517 - protein, 219 aa, Artificial Sequence; identical to SEQ ID NO: 501
  Synthetic Construct

SEQ ID NO: 518 - protein, 438 aa, Artificial Sequence
  Synthetic Construct
QVQLVQSGAEVVKPGSSVKVSCEASGFTFTDSVITWVRQRPGQGLEWIGEIYPGSGNFYYNEKFQGRVTITADKSTSTAYMELSSLRSEDTAVYFCAMRRSSWGQGTLVTVSSASTKGPSVFPLAPSSKSTSGGTAALGCLVKDYFPEPVTVSWNSGALTSGVHTFPAVLQSSGSLSSVVTVPSSSLGTQTYICNVNHKPSNTKVDKKVEPKSCDKTHTCPPCPAPELLGGPSVFLFPPKPKDTLMISRTPEVTCVVVDVSHEDPEVKFNWYVDGVEVHNAKTKPREEQYNNASRVVSVLTVLHQDWLNGKEYKCKVSNKALPAPIEKTISKAKGQPREPQVYTLPPSRDELTKNQVSLTCLVKGFYPSDIAVEWESNGQPENNYKTTPPVLDSDGSFFKRLTVDKSRWQQGNVFSCSVMHEALHNHYTQKSLSLSPG

SEQ ID NO: 519 - protein, 443 aa, Artificial Sequence
  Synthetic Construct
EVQLVESGGGLVKPGGSLRLSCAASGFTFSSYTMSWVRQAPGKGLEWVASISSSGSNTYYPDSVKGRFTISRDNAKNNLYLQMNSLRAEDTALYYCARFDYGSSLDSWGQGTLLTVSSASTKGPSVFPLAPSSKSTSGGTAALGCLVKDYFPEPVTVSWNSGALTSGVHTFPAVLQSSGSLSSVVTVPSSSLGTQTYICNVNHKPSNTKVDKKVEPKSCDKTHTCPPCPAPELLGGPSVFLFPPKPKDTLMISRTPEVTCVVVDVSHEDPEVKFNWYVDGVEVHNAKTKPREEQYNNSARVVSVLTVLHQDWLNGKEYKCKVSNKALPAPIEKTISKAKGQPREPQVYTLPPSRDELTKNQVSLTCLVKGFYPSDIAVEWESNGQPENNYKTTPPVLDSDGSFLKKLTVDKSRWQQGNVFSCSVMHEALHNHYTQKSLSLSPG

SEQ ID NO: 520 - protein, 219 aa, Artificial Sequence; identical to SEQ ID NO: 501
  Synthetic Construct

SEQ ID NO: 521 - protein, 214 aa, Artificial Sequence
  Synthetic Construct
EIVLTQSPDFLSVTPKEKVTLTCRASQSISNNLHWYQQKSDQSPKLLIKYASQSISGIPSRFSGSGSGTDFTLTINSVEAEDAATYFCQQSKSWPRTFGGGTKLEIKRTVAAPSVFIFPPSDEQLKSGTASVVCLLNNFYPREAKVQWKVDNALQSGNSQESVTEQDSKDSTYSLSSTLTLSKADYEKHKVYACEVTHQGLSSPVTKSFNRGEC

SEQ ID NO: 522 - protein, 566 aa, Artificial Sequence
  Synthetic Construct
QVQLVQSGAEVVKPGSSVKVSCEASGFTFTDSVITWVRQRPGQGLEWIGEIYPGSGNFYYNEKFQGRVTITADKSTSTAYMELSSLRSEDTAVYFCAMRRSSWGQGTLVTVSSGGGGSGGGGSEVQLVESGGGLVKPGGSLRLSCAASGFTFSSYTMSWVRQAPGKGLEWVASISSSGSNTYYPDSVKGRFTISRDNAKNNLYLQMNSLRAEDTALYYCARFDYGSSLDSWGQGTLLTVSSASTKGPSVFPLAPSSKSTSGGTAALGCLVKDYFPEPVTVSWNSGALTSGVHTFPAVLQSSGSLSSVVTVPSSSLGTQTYICNVNHKPSNTKVDKKVEPKSCDKTHTCPPCPAPELLGGPSVFLFPPKPKDTLMISRTPEVTCVVVDVSHEDPEVKFNWYVDGVEVHNAKTKPREEQYNNASRVVSVLTVLHQDWLNGKEYKCKVSNKALPAPIEKTISKAKGQPREPQVYTLPPSRDELTKNQVSLTCLVKGFYPSDIAVEWESNGQPENNYKTTPPVLDSDGSFFKKLTVDKSRWQQGNVFSCSVMHEALHNHYTQKSLSLSPG

SEQ ID NO: 523 - protein, 336 aa, Artificial Sequence
  Synthetic Construct
DVVMTQTPLSLSVTPGQPASISCKSSQTIVHSNSKTYLEWYLQKPGQSPQLLIYKVSSRFSGVPDRFSGSGSGTDFTLKISRVEAEDVGVYYCFQGSHVPLTFGQGTKLEIKGGGGSGGGGSEIVLTQSPDFLSVTPKEKVTLTCRASQSISNNLHWYQQKSDQSPKLLIKYASQSISGIPSRFSGSGSGTDFTLTINSVEAEDAATYFCQQSKSWPRTFGGGTKLEIKRTVAAPSVFIFPPSDEQLKSGTASVVCLLNNFYPREAKVQWKVDNALQSGNSQESVTEQDSKDSTYSLSSTLTLSKADYEKHKVYACEVTHQGLSSPVTKSFNRGEC

SEQ ID NO: 524 - protein, 438 aa, Artificial Sequence
  Synthetic Construct
QVQLVQSGAEVVKPGSSVKVSCEASGFTFTDSVITWVRQRPGQGLEWIGEIYPGSGNFYYNEKFQGRVTITADKSTSTAYMELSSLRSEDTAVYFCAMRRSSWGQGTLVTVSSASTKGPSVCPLAPSSKSTSGGTAALGCLVKDYFPEPVTVSWNSGALTSGVHTFPAVLQSSGSLSSVVTVPSSSLGTQTYICNVNHKPSNTKVDKKVEPKSVDKTHTCPPCPAPELLGGPSVFLFPPKPKDTLMISRTPEVTCVVVDVSHEDPEVKFNWYVDGVEVHNAKTKPREEQYNNASRVVSVLTVLHQDWLNGKEYKCKVSNKALPAPIEKTISKAKGQPREPQVYTLPPCRDELTKNQVSLWCLVKGFYPSDIAVEWESNGQPENNYKTTPPVLDSDGSFFKKLTVDKSRWQQGNVFSCSVMHEALHNHYTQKSLSLSPG

SEQ ID NO: 525 - protein, 445 aa, Artificial Sequence
  Synthetic Construct
EVQLVESGGGLVKPGGSLRLSCAASGFTFSSYTMSWVRQAPGKGLEWVASISSSGSNTYYPDSVKGRFTISRDNAKNNLYLQMNSLRAEDTALYYCARFDYGSSLDSWGQGTLLTVSSASTKGPSVFPLAPSSKSTSGGTAALGCLVKDYFPEPVTVSWNSGALTSGVHTFPAVLQSSGSLSSVVTVPSSSLGTQTYICNVNHKPSNTKVDKKVEPKSCDKTHTCPPCPAPELLGGPSVFLFPPKPKDTLMISRTPEVTCVVVDVSHEDPEVKFNWYVDGVEVHNAKTKPREEQYNNASRVVSVLTVLHQDWLNGKEYKCKVSNKALPAPIEKTISKAKGQPREPQVCTLPPSRDELTKNQVSLSCAVKGFYPSDIAVEWESNGQPENNYKTTPPVLDSDGSFFLVSKLTVDKSRWQQGNVFSCSVMHEALHNRFTQKSLSLSPG

SEQ ID NO: 526 - protein, 219 aa, Artificial Sequence
  Synthetic Construct
DVVMTQTPLSLSVTPGQPASISCKSSQTIVHSNSKTYLEWYLQKPGQSPQLLIYKVSSRFSGVPDRFSGSGSGTDFTLKISRVEAEDVGVYYCFQGSHVPLTFGQGTKLEIKRTVAAPSVFIFPPCDEQLKSGTASVVCLLNNFYPREAKVQWKVDNALQSGNSQESVTEQDSKDSTYSLSSTLTLSKADYEKHKVYACEVTHQGLSSPVTKSFNRGEV

SEQ ID NO: 527 - protein, 214 aa, Artificial Sequence
  Synthetic Construct
EIVLTQSPDFLSVTPKEKVTLSCRASQSISNYLHWYQQKSDQSPKLLIKYASQSISGIPSRFSGSGSGTDFTLSINSVEAEDAATYFCQQSKSWPRTFGGGTKLEIKRTVAAPSVFIFPPSDEQLKSGTASVVCLLNNFYPREAKVQWKVDNALQSGNSQESVTEQDSKDSTYSLSSTLTLSKADYEKHKVYACEVTHQGLSSPVTKSFNRGEC

SEQ ID NO: 528 - protein, 566 aa, Artificial Sequence; identical to SEQ ID NO: 522
  Synthetic Construct

SEQ ID NO: 529 - protein, 336 aa, Artificial Sequence
  Synthetic Construct
DVVMTQTPLSLSVTPGQPASISCKSSQTIVHSNSKTYLEWYLQKPGQSPQLLIYKVSSRFSGVPDRFSGSGSGTDFTLKISRVEAEDVGVYYCFQGSHVPLTFGQGTKLEIKGGGGSGGGGSEIVLTQSPDFLSVTPKEKVTLSCRASQSISNYLHWYQQKSDQSPKLLIKYASQSISGIPSRFSGSGSGTDFTLSINSVEAEDAATYFCQQSKSWPRTFGGGTKLEIKRTVAAPSVFIFPPSDEQLKSGTASVVCLLNNFYPREAKVQWKVDNALQSGNSQESVTEQDSKDSTYSLSSTLTLSKADYEKHKVYACEVTHQGLSSPVTKSFNRGEC

SEQ ID NO: 530 - protein, 559 aa, Artificial Sequence
  Synthetic Construct
QVQLVQSGAEVVKPGSSVKVSCEASGFTFTDSVITWVRQRPGQGLEWIGEIYPGSGNFYYNEKFQGRVTITADKSTSTAYMELSSLRSEDTAVYFCAMRRSSWGQGTLVTVSSSEVQLVESGGGLVKPGGSLRLSCAASGFTFSSYTMSWVRQAPGKGLEWVASISSSGSNTYYPDSVKGRFTISRDNAKNNLYLQMNSLRAEDTALYYCARFDYGSSLDSWGQGTLLTVSSRTASTKGPSVFPLAPSSKSTSGGTAALGCLVKDYFPEPVTVSWNSGALTSGVHTFPAVLQSSGSLSSVVTVPSSSLGTQTYICNVNHKPSNTKVDKKVEPKSCDKTHTCPPCPAPELLGGPSVFLFPPKPKDTLMISRTPEVTCVVVDVSHEDPEVKFNWYVDGVEVHNAKTKPREEQYNNASRVVSVLTVLHQDWLNGKEYKCKVSNKALPAPIEKTISKAKGQPREPQVYTLPPSRDELTKNQVSLTCLVKGFYPSDIAVEWESNGQPENNYKTTPPVLDSDGSFFKKLTVDKSRWQQGNVFSCSVMHEALHNHYTQKSLSLSPG

SEQ ID NO: 531 - protein, 338 aa, Artificial Sequence
  Synthetic Construct
EIVLTQSPDFLSVTPKEKVTLTCRASQSIGNNLHWYQQKSDQSPKLLIKYASQSISGIPSRFSGSGSGTDFTLTINSVEAEDAATYFCQQSKSWPRTFGGGTKLEIKGQPKAAPDVVMTQTPLSLSVTPGQPASISCRSSQTIVHSNSKTYLEWYLQKPGQSPQLLIYKVSNRFSGVPDRFSGSGSGTDFTLKISRVEAEDVGVYYCFQGSHVPLTFGAGTKLEIKTKGPSRTVAAPSVFIFPPSDEQLKSGTASVVCLLNNFYPREAKVQWKVDNALQSGNSQESVTEQDSKDSTYSLSSTLTLSKADYEKHKVYACEVTHQGLSSPVTKSFNRGEC

SEQ ID NO: 532 - protein, 559 aa, Artificial Sequence
  Synthetic Construct
QVQLVQSGAEVVKPGSSVKVSCEASGFTFTDSVITWVRQRPGQGLEWIGEIYPGSGNFYYNEKFQGRVTITADKSTSTAYMELSSLRSEDTAVYFCAMRRSSWGQGTLVTVSSSEVQLVESGGGLVQPGGSLRLSCAASGFTFSSYTMSWVRQAPGKGLEWVATISSSGDNTYYPDSVKGRFTISRDNSKNTLYLQMSSLRAEDTALYYCARFDYGSSLDSWGQGTTLTVSSRTASTKGPSVFPLAPSSKSTSGGTAALGCLVKDYFPEPVTVSWNSGALTSGVHTFPAVLQSSGSLSSVVTVPSSSLGTQTYICNVNHKPSNTKVDKKVEPKSCDKTHTCPPCPAPELLGGPSVFLFPPKPKDTLMISRTPEVTCVVVDVSHEDPEVKFNWYVDGVEVHNAKTKPREEQYNNASRVVSVLTVLHQDWLNGKEYKCKVSNKALPAPIEKTISKAKGQPREPQVYTLPPSRDELTKNQVSLTCLVKGFYPSDIAVEWESNGQPENNYKTTPPVLDSDGSFFKKLTVDKSRWQQGNVFSCSVMHEALHNHYTQKSLSLSPG

SEQ ID NO: 533 - protein, 338 aa, Artificial Sequence
  Synthetic Construct
EIVLTQSPDFLSVTPGEKVTLTCRASQSISNYLHWYQQKSDQSPKLLIKYASQSISGVPSRFSGSGSGTDFTLTISSVEAEDFATYFCQQSKSWPRTFGGGTKLEIKGQPKAAPDVVMTQTPLSLSVTPGQPASISCRSSQTIVHSNSKTYLEWYLQKPGQSPQLLIYKVSNRFSGVPDRFSGSGSGTDFTLKISRVEAEDVGVYYCFQGSHVPLTFGAGTKLEIKTKGPSRTVAAPSVFIFPPSDEQLKSGTASVVCLLNNFYPREAKVQWKVDNALQSGNSQESVTEQDSKDSTYSLSSTLTLSKADYEKHKVYACEVTHQGLSSPVTKSFNRGEC

SEQ ID NO: 534 - protein, 5 aa, Artificial Sequence
  Synthetic Construct
DKTHT